European Patent Specification EP 3 448 417 B1, published November 12, 2025. Title: INSULIN DIMER-INCRETIN CONJUGATES. Applicant: Merck Sharp & Dohme Corp. Palani, Anandan Yang, ZhiQiang Yan, Lin Lin, Songnian Huo, Pei Nargund, Ravi. The sequence listing filed with the application follows.

SEQUENCE LISTING (141 sequences)

SEQ ID NO: 1 - protein, 29 aa, Artificial Sequence
  Glucagon-derived peptide
HSQGTFTSDYSKYLDERAAQDFVQWLLDT

SEQ ID NO: 2 - protein, 31 aa, Artificial Sequence
  Peptide
  PEPTIDE (1)..(31): C-terminal amino acid optionally is linked to a protecting group or amidated
  PEPTIDE (1)..(31): with the proviso that either X10 is a Lysine residue conjugatedto lipid moiety and one of X20, X21, X24, X30, or X31 comprises the azide group or X20 is a Lysine residue conjugated lipid moiety and one of X21, X24, X30, or X31 comprises the azide group
  MISC_FEATURE (2)..(2): Xaa is amionisobutyric acid (Aib), Gly, D-Serine (s), alpha-methyl Serine (?MS), or alpha-methyl D-Serine (alpha-Ms)
  MISC_FEATURE (3)..(3): Xaa is Val, Glu or Asp
  MISC_FEATURE (9)..(9): Xaa is Asp or alpha-methyl Aspartic acid (alpha-MD)
  MISC_FEATURE (10)..(10): Xaa is Tyr or Lys conjugated to a lipid moiety
  MISC_FEATURE (12)..(12): Xaa is Lysine, Leucine, or Serine
  MISC_FEATURE (14)..(14): Xaa is Leu of alpha-methyl Leucine (alpha-ML)
  MISC_FEATURE (16)..(16): Xaa is Glutamic acid, Asparagine, Serine, Alanine, or Aib
  MISC_FEATURE (17)..(17): Xaa is Arginine or Lysine
  MISC_FEATURE (18)..(18): Xaa is Alanine or Arginine
  MISC_FEATURE (20)..(20): Xaa is Glutamine or Lysine conjugated via its epsilon amino group to a non-peptide linker comprising a terminal azide group or to a fatty acid or fatty diacid
  MISC_FEATURE (21)..(21): Xaa is Aspartic acid, ?MD, Azidonorleucine (Norleucine conjugated via its epsilon carbon to an azide group (Nle(?N3))), or Lysine conjugated via its epsilon amino group to a non-peptide linker comprising a terminal azide group
  MISC_FEATURE (22)..(22): Xaa is Phe or alpha-MF
  MISC_FEATURE (24)..(24): Xaa is Glutamine, Nle(epsilon-N3), or Lysine conjugated via its epsilon amino group to a non-peptide linker comprising a terminal azide group
  MISC_FEATURE (25)..(25): Xaa is Tryptophan or alpha-methyl Tryptophan (alpha-MW);
  MISC_FEATURE (26)..(26): Xaa is Leucine or alpha-ML
  MISC_FEATURE (27)..(27): Xaa is Methionine, Leucine, Methionine sulfoxide, or L-methionine sulphone (2)
  MISC_FEATURE (28)..(28): Xaa is Aspartic acid, Alanine, Lysine, Asparagine, gamma-Glu, Glutamine, or alpha-MD
  MISC_FEATURE (29)..(29): Xaa is Threonine or Glycine
  MISC_FEATURE (30)..(30): Xaa is Arginine, Lysine, or Nle(epsilonN3), or Xaa is absent
  MISC_FEATURE (31)..(31): Xaa is Glycine, gamma-Glu, Nle(epsilon-N3), or Lysine conjugated via its epsilon amino group to a non-peptide linker comprising a terminal azide group, or Xaa is absent
HXXGTFTSXXSXYXDXXXAXXXVXXXXXXXX

SEQ ID NO: 3 - protein, 31 aa, Artificial Sequence; identical to SEQ ID NO: 2
  Peptide
  PEPTIDE (1)..(31): C-terminal amino acid optionally is linked to a protecting group or amidated
  PEPTIDE (1)..(31): with proviso that either X10 is a Lysine residue conjugated the lipid moiety and one of X20, X21, X24, X30, or X31 comprises the alkyne group or X20 is a Lysine residue conjugated to the lipid moiety and one of X21, X24, X30, or X31 comprises the alkyne
  MISC_FEATURE (2)..(2): Xaa is aminoisobutyric acid (Aib), D-Serine (s), or alpha-methyl Serine (alpha-MS)
  MISC_FEATURE (3)..(3): Xaa is Val, Glu, or Asp
  MISC_FEATURE (9)..(9): Xaa is Asp or alpha-methyl Aspartic acid (alpha-MD)
  MISC_FEATURE (10)..(10): Xaa is Tyr or Lys conjugated to a lipid moiety
  MISC_FEATURE (12)..(12): Xaa is Lysine, Leucine, or Serine
  MISC_FEATURE (14)..(14): Xaa is Leu or alpha-methyl Leucine (alpha-ML)
  MISC_FEATURE (16)..(16): Xaa is Glutamic acid, Asparagine, Serine, Alanine, or Aib
  MISC_FEATURE (17)..(17): Xaa is Arginine or Lysine
  MISC_FEATURE (18)..(18): Xaa is Alanine or Arginine
  MISC_FEATURE (20)..(20): Xaa is Glutamine or Lysine conjugated via its epsilon amino group to a non-peptide linker comprising a terminal alkyne group or to a fatty acid or fatty diacid
  MISC_FEATURE (21)..(21): Xaa is Aspartic acid, alpha-MD, Alkynylnorleucine (Norleucine conjugated via its epsilon carbon to an alkyne group (Nle(epsilon-alkyne))), or Lysine conjugated via its epsilon amino group to a non-peptide linker comprising a terminal alkyne
  MISC_FEATURE (22)..(22): Xaa is Phe or alpha-methyl Phenylalanine (alpha-MF)
  MISC_FEATURE (24)..(24): Xaa is Glutamine, Nle(epsilon-alkyne), or Lysine conjugated via its epsilon amino group to a non-peptide linker comprising a terminal alkyne group
  MISC_FEATURE (25)..(25): Xaa is Tryptophan or alpha-methyl Tryptophan (alpha-MW)
  MISC_FEATURE (26)..(26): Xaa is Leucine or alpha-ML
  MISC_FEATURE (27)..(27): Xaa is Methionine, Leucine, methionine sulfoxide, or L-methionine sulphone (2)
  MISC_FEATURE (28)..(28): Xaa is Aspartic acid, Alanine, Lysine, Asparagine, gamma-Glu, Glutamine, or alpha-MD
  MISC_FEATURE (29)..(29): Xaa is Threonine or Glycine
  MISC_FEATURE (30)..(30): Xaa is Arginine, Lysine, or Nle(epsilon-alkyne), or Xaa is absent
  MISC_FEATURE (31)..(31): Xaa is Glycine, ?Glu, Nle(epsilon-alkyne), or Lysine conjugated via its epsilon amino group to a non-peptide linker comprising a terminal alkyne group, or Xaa is absent

SEQ ID NO: 4 - protein, 31 aa, Artificial Sequence
  Peptide
  PEPTIDE (1)..(31): C-terminal amino acid optionally is linked to a protecting group or amidated
  PEPTIDE (1)..(31): with proviso that either X10 is a Lysine residue conjugated lipid moiety and one of X20, X21, X24, X30, or X31 comprises the azide group or X20 is a Lysine residue conjugated lipid moiety and one of X21, X24, X30, or X31 comprises the azide group
  MISC_FEATURE (2)..(2): Xaa is aminoisobutyric acid (Aib), D-Serine (s), or alpha-methyl Serine (alpha-MS)
  MISC_FEATURE (9)..(9): Xaa is Asp or alpha-methyl Aspartic acid (alpha-MD)
  MISC_FEATURE (10)..(10): Xaa is Tyr or Lys conjugated to a lipid moiety
  MISC_FEATURE (12)..(12): Xaa is Lysine, Leucine, or Serine
  MISC_FEATURE (16)..(16): Xaa is Glutamic acid, Asparagine, Serine, Alanine, or Aib
  MISC_FEATURE (17)..(17): Xaa is Arginine or Lysine
  MISC_FEATURE (18)..(18): Xaa is Alanine or Arginine
  MISC_FEATURE (20)..(20): Xaa is Glutamine or Lysine conjugated via its epsilon amino group to a non-peptide linker comprising a terminal azide group or to a fatty acid or fatty diacid
  MISC_FEATURE (21)..(21): Xaa is Aspartic acid, alpha-MD, Azidonorleucine (Norleucine conjugated via its epsilon carbon to an azide group (Nle(epsilon-N3))), or Lysine conjugated via its epsilon amino group to a non-peptide linker comprising a terminal azide group
  MISC_FEATURE (22)..(22): Xaa is Phe or alpha-methyl Phenylalanine (alpha-MF)
  MISC_FEATURE (24)..(24): Xaa is Glutamine, Nle(epsilon-N3), or Lysine conjugated via its epsilon amino group to a non-peptide linker comprising a terminal azide group
  MISC_FEATURE (25)..(25): Xaa is Tryptophan or alpha-methyl Tryptophan (alpha-MW)
  MISC_FEATURE (26)..(26): Xaa is Leucine or alpha-ML
  MISC_FEATURE (27)..(27): Xaa is Methionine, Leucine, methionine sulfoxide, or L-methionine sulphone (2)
  MISC_FEATURE (28)..(28): Xaa is Aspartic acid, Alanine, Lysine, Asparagine, ?Glu, Glutamine, or alpha-MD
  MISC_FEATURE (29)..(29): Xaa is Threonine or Glycine
  MISC_FEATURE (30)..(30): Xaa is Arginine, Lysine, or Nle(epsilon-N3), or X30 is absent
  MISC_FEATURE (31)..(31): Xaa is Glycine, gamma-Glu, Nle(epsilon-N3), or Lysine conjugated via its epsilon amino group to a non-peptide linker comprising a terminal azide group, or X31 is absent
HXQGTFTSXXSXYXDXXXAXXXVXXXXXXXX

SEQ ID NO: 5 - protein, 31 aa, Artificial Sequence; identical to SEQ ID NO: 4
  Peptide
  PEPTIDE (1)..(31): C-terminal amino acid optionally is linked to a protecting group or amidated
  PEPTIDE (1)..(31): with the proviso that either X10 is a Lysine residue conjugated lipid moiety and one of X20, X21, X24, X30, or X31 comprises the alkyne group or X20 is a Lysine residue conjugated lipid moiety and one of X21, X24, X30, or X31 comprises the alkyne group
  MISC_FEATURE (2)..(2): Xaa is aminoisobutyric acid (Aib), D-Serine (s), or alpha-methyl Serine (alpha-MS)
  MISC_FEATURE (9)..(9): Xaa is Asp or alpha-methyl Aspartic acid (alpha-MD)
  MISC_FEATURE (10)..(10): Xaa is Tyr or Lys conjugated to a lipid moiety
  MISC_FEATURE (12)..(12): Xaa is Lysine, Leucine, or Serine
  MISC_FEATURE (14)..(14): Xaa is Leu of alpha-methyl Leucine (alpha-ML)
  MISC_FEATURE (16)..(16): Xaa is Glutamic acid, Asparagine, Serine, Alanine, or Aib
  MISC_FEATURE (17)..(17): Xaa is Arginine or Lysine
  MISC_FEATURE (18)..(18): Xaa is Alanine or Arginine
  MISC_FEATURE (20)..(20): Xaa is Glutamine or Lysine conjugated via its epsilon amino group to a non-peptide linker comprising a terminal alkyne group or to a fatty acid or fatty diacid
  MISC_FEATURE (21)..(21): Xaa is Aspartic acid, alpha-MD, Alkynylnorleucine (Norleucine conjugated via its epsilon carbon to an alkyne group (Nle(epsilon-alkyne))), or Lysine conjugated via its epsilon amino group to a non-peptide linker comprising a terminal alkyne
  MISC_FEATURE (22)..(22): Xaa is Phe or alpha-methyl Phenylalanine (alpha-MF)
  MISC_FEATURE (24)..(24): Xaa is Glutamine, Nle(epsilon-alkyne), or Lysine conjugated via its epsilon amino group to a non-peptide linker comprising a terminal alkyne group
  MISC_FEATURE (25)..(25): Xaa is Tryptophan or alpha-methyl Tryptophan (alpha-MW)
  MISC_FEATURE (26)..(26): Xaa is Leucine or alpha-ML
  MISC_FEATURE (27)..(27): Xaa is Methionine, Leucine, methionine sulfoxide, or L-methionine sulphone (2)
  MISC_FEATURE (28)..(28): Xaa is Aspartic acid, Alanine, Lysine, Asparagine, gamma-Glu, Glutamine, or alpha-MD
  MISC_FEATURE (29)..(29): Xaa is Threonine or Glycine
  MISC_FEATURE (30)..(30): Xaa is Arginine, Lysine, or Nle(epsilon-alkyne), or Xaa is absent and
  MISC_FEATURE (31)..(31): Xaa is Glycine, gamma-Glu, Nle(epsilon-alkyne), or Lysine conjugated via its epsilon amino group to a non-peptide linker comprising a terminal alkyne group, or Xaa is absent

SEQ ID NO: 6 - protein, 31 aa, Artificial Sequence
  Peptide
  MISC_FEATURE (1)..(1): Xaa is Tyrosine, Phenylalanine, Tryptophan, or other amino acid with an aromatic group
  PEPTIDE (1)..(31): C-terminal amino acid optionally is linked to a protecting group or amidated
  PEPTIDE (1)..(31): with the proviso that either X10 is a Lysine residue conjugated lipid moiety and one of X20, X21, X24, X30, or X31 comprises the azide group or X20 is a Lysine residue conjugated lipid moiety and one of X21, X24, X30, or X31 comprises the azide group
  MISC_FEATURE (2)..(2): Xaa is amionisobutyric acid (Aib), Gly, D-Serine (s), or alpha-methyl Serine (alpha-MS)
  MISC_FEATURE (3)..(3): Xaa is Val, Glu, or Asp
  MISC_FEATURE (9)..(9): Xaa is Asp or alpha-methyl Aspartic acid (alpha-MD)
  MISC_FEATURE (10)..(10): X10 is Tyr or Lys conjugated to a lipid moiety
  MISC_FEATURE (12)..(12): Xaa is Isoleucine, Lysine, Leucine, or Serine
  MISC_FEATURE (14)..(14): Xaa is Leu of alpha-methyl Leucine (alpha-ML)
  MISC_FEATURE (16)..(16): Xaa is Glutamic acid, Asparagine, Serine, Alanine, or Aib
  MISC_FEATURE (17)..(17): Xaa is Arginine or Lysine
  MISC_FEATURE (18)..(18): Xaa is Alanine or Arginine
  MISC_FEATURE (20)..(20): Xaa is Glutamine or Lysine conjugated via its epsilon amino group to a non-peptide linker comprising a terminal azide group or to a fatty acid or fatty diacid
  MISC_FEATURE (21)..(21): Xaa is Aspartic acid, alpha-MD, Azidonorleucine (Norleucine conjugated via its epsilon carbon to an azide group (Nle(epsilon-N3))), or Lysine conjugated via its epsilon amino group to a non-peptide linker comprising a terminal azide group
  MISC_FEATURE (22)..(22): Xaa is Phe or alpha-methyl Phenylalanine (alpha-MF),
  MISC_FEATURE (24)..(24): Xaa is Glutamine, Nle(epsilon-N3), or Lysine conjugated via its epsilon amino group to a non-peptide linker comprising a terminal azide group
  MISC_FEATURE (25)..(25): Xaa is Tryptophan or alpha-methyl Tryptophan (alpha-MW)
  MISC_FEATURE (26)..(26): Xaa is Leucine or alpha-ML
  MISC_FEATURE (27)..(27): Xaa is Met, Leucine, methionine sulfoxide, or L-methionine sulphone (2)
  MISC_FEATURE (28)..(28): Xaa is Aspartic acid, Alanine, Lysine, Asparagine, gamma-Glu, Glutamine, or alpha-MD
  MISC_FEATURE (29)..(29): Xaa is Threonine or Glycine
  MISC_FEATURE (30)..(30): Xaa is Arginine, Lysine, or Nle(epsilon-N3), or Xaa is absent and
  MISC_FEATURE (31)..(31): Xaa is Glycine, gamma-Glu, Nle(epsilon-N3), or Lysine conjugated via its epsilon amino group to a non-peptide linker comprising a terminal azide group, or Xaa is absent
XXXGTFTSXXSXYXDXXXAXXXVXXXXXXXX

SEQ ID NO: 7 - protein, 31 aa, Artificial Sequence; identical to SEQ ID NO: 6
  Peptide
  MISC_FEATURE (1)..(1): Xaa is Tyrosine, Phenylalanine, Tryptophan, or other amino acid with an aromatic group
  PEPTIDE (1)..(31): C-terminal amino acid optionally is linked to a protecting group or amidated
  PEPTIDE (1)..(31): with the proviso that either X10 is a Lysine residue conjugated to  lipid moiety and one of X20, X21, X24, X30, or X31 comprises the alkyne group or X20 is a Lysine residue conjugated to lipid moiety and one of X21, X24, X30, or X31 comprises the alkyne
  MISC_FEATURE (2)..(2): Xaa is aminoisobutyric acid (Aib), D-Serine (s), or alpha-methyl Serine (alpha-MS)
  MISC_FEATURE (3)..(3): Xaa is Val, Glu, or Asp
  MISC_FEATURE (9)..(9): Xaa is Asp or alpha-methyl Aspartic acid (alpha-MD)
  MISC_FEATURE (10)..(10): Xaa is Tyr or Lys conjugated to a lipid moiety
  MISC_FEATURE (12)..(12): Xaa is Isoleucine, Lysine, Leucine, or Serine
  MISC_FEATURE (14)..(14): Xaa is Leu of alpha-methyl Leucine (alpha-ML)
  MISC_FEATURE (16)..(16): Xaa is Glutamic acid, Asparagine, Serine, Alanine, or Aib
  MISC_FEATURE (17)..(17): Xaa is Arginine or Lysine
  MISC_FEATURE (18)..(18): Xaa is Alanine or Arginine
  MISC_FEATURE (20)..(20): Xaa is Glutamine or Lysine conjugated via its epsilon amino group to a non-peptide linker comprising a terminal alkyne group or to a fatty acid or fatty diacid
  MISC_FEATURE (21)..(21): Xaa is Aspartic acid, alpha-MD, Alkynylnorleucine (Norleucine conjugated via its epsilon carbon to an alkyne group (Nle(epsilon-alkyne))), or Lysine conjugated via its epsilon amino group to a non-peptide linker comprising a terminal alkyne
  MISC_FEATURE (22)..(22): Xaa is Phe or alpha-methyl Phenylalanine (alpha-MF),
  MISC_FEATURE (24)..(24): Xaa is Glutamine, Nle(epsilon-alkyne), or Lysine conjugated via its epsilon amino group to a non-peptide linker comprising a terminal alkyne group
  MISC_FEATURE (26)..(26): Xaa is Leucine or alpha-ML
  MISC_FEATURE (27)..(27): Xaa is Methionine, Leucine, methionine sulfoxide, or L-methionine sulphone (2)
  MISC_FEATURE (28)..(28): Xaa is Aspartic acid, Alanine, Lysine, Asparagine, gamma-Glu, Glutamine, or alpha-MD
  MISC_FEATURE (29)..(29): Xaa is Threonine or Glycine
  MISC_FEATURE (30)..(30): Xaa is Arginine, Lysine, or Nle(epsilon-alkyne), or Xaa is absent and
  MISC_FEATURE (31)..(31): Xaa is Glycine, gamma-Glu, Nle(epsilon-alkyne), or Lysine conjugated via its epsilon amino group to a non-peptide linker comprising a terminal alkyne group, or Xaa is absent and

SEQ ID NO: 8 - protein, 31 aa, Artificial Sequence
  Peptide
  MISC_FEATURE (1)..(1): Xaa is Tyrosine, Phenylalanine, Tryptophan, or other amino acid with an aromatic group
  PEPTIDE (1)..(31): C-terminal amino acid optionally is linked to a protecting group or amidated
  PEPTIDE (1)..(31): with the proviso that either X10 is a Lysine residue conjugated to  lipid moiety and one of X20, X21, X24, X30, or X31 comprises the azide group or X20 is a Lysine residue conjugated to  lipid moiety and one of X21, X24, X30, or X31 comprises the azide group
  MISC_FEATURE (2)..(2): Xaa is amionisobutyric acid (Aib), Gly, D-Serine (s), or alpha-methyl Serine (alpha-MS)
  MISC_FEATURE (10)..(10): Xaa is Tyr or Lys conjugated to a lipid moiety
  MISC_FEATURE (12)..(12): Xaa is Isoleucine, Lysine, Leucine, or Serine
  MISC_FEATURE (14)..(14): Xaa is Leu of alpha-methyl Leucine (alpha-ML)
  MISC_FEATURE (16)..(16): Xaa is Glutamic acid, Asparagine, Serine, Alanine, or Aib
  MISC_FEATURE (17)..(17): Xaa is Glutamic acid, Asparagine, Serine, Alanine, or Aib
  MISC_FEATURE (17)..(17): Xaa is Arginine or Lysine
  MISC_FEATURE (18)..(18): Xaa is Alanine or Arginine
  MISC_FEATURE (20)..(20): Xaa is Glutamine or Lysine conjugated via its epsilon amino group to a non-peptide linker comprising a terminal azide group or to a fatty acid or fatty diacid
  MISC_FEATURE (21)..(21): Xaa is Aspartic acid, alpha-MD, Azidonorleucine (Norleucine conjugated to an azide group (Nle(epsilonN3))), or Lysine conjugated via to a non-peptide linker comprising a terminal azide group
  MISC_FEATURE (22)..(22): Xaa is Phe or alpha-methyl Phenylalanine (alpha-MF)
  MISC_FEATURE (24)..(24): Xaa is Glutamine, Nle(epsilonN3), or Lysine conjugated via its epsilon amino group to a non-peptide linker comprising a terminal azide group
  MISC_FEATURE (25)..(25): Xaa is Tryptophan or alpha-methyl Tryptophan (alpha-MW)
  MISC_FEATURE (26)..(26): Xaa is Leucine or alpha-ML
  MISC_FEATURE (27)..(27): Xaa is methionine, Leucine, methionine sulfoxide, or L-methionine sulphone (2)
  MISC_FEATURE (28)..(28): Xaa is Aspartic acid, Alanine, Lysine, Asparagine, gamma-Glu, Glutamine, or alpha-MD
  MISC_FEATURE (29)..(29): Xaa is Threonine or Glycine
  MISC_FEATURE (30)..(30): Xaa is Arginine, Lysine, or Nle(epsilonN3), or Xaa is absent and
  MISC_FEATURE (31)..(31): XAA is Glycine, gamma-Glu, Nle(epsilonN3), or Lysine conjugated via its epsilon amino group to a non-peptide linker comprising a terminal azide group, or XAA is absent and
XXQGTFTSXXSXYXDXXXAXXXVXXXXXXXX

SEQ ID NO: 9 - protein, 31 aa, Artificial Sequence
  Peptide
  MISC_FEATURE (1)..(1): Xaa is Tyrosine, Phenylalanine, Tryptophan, or other amino acid with an aromatic group
  PEPTIDE (1)..(31): C-terminal amino acid optionally is linked to a protecting group or amidated
  PEPTIDE (1)..(31): with the proviso that either X10 is a Lysine residue conjugated to  lipid moiety and one of X20, X21, X24, X30, or X31 comprises the alkyne group or X20 is a Lysine residue conjugated to  lipid moiety and one of X21, X24, X30, or X31 comprises the alkyne
  MISC_FEATURE (2)..(2): X2 is aminoisobutyric acid (Aib), D-Serine (s), or alpha-methyl Serine (alpha-MS)
  MISC_FEATURE (9)..(9): Xaa is Asp or alpha-methyl Aspartic acid (alpha-MD)
  MISC_FEATURE (10)..(10): X10 is Tyr or Lys conjugated to a lipid moiety
  MISC_FEATURE (12)..(12): Xaa is Isoleucine, Lysine, Leucine, or Serine
  MISC_FEATURE (14)..(14): Xaa is Leu of alpha-methyl Leucine (alpha-ML)
  MISC_FEATURE (16)..(16): Xaa is Glutamic acid, Asparagine, Serine, Alanine, or Aib
  MISC_FEATURE (17)..(17): Xaa is Arginine or Lysine
  MISC_FEATURE (18)..(18): Xaa is Alanine or Arginine
  MISC_FEATURE (20)..(20): Xaa is Glutamine or Lysine conjugated via its epsilon amino group to a non-peptide linker comprising a terminal alkyne group or to a fatty acid or fatty diacid
  MISC_FEATURE (21)..(21): Xaa is Aspartic acid, alpha-MD, Alkynylnorleucine (Norleucine conjugated via its epsilon carbon to an alkyne group (Nle(epsilon-alkyne))), or Lysine conjugated via its epsilon amino group to a non-peptide linker comprising a terminal alkyne
  MISC_FEATURE (22)..(22): Xaa is Phe or alpha-methyl Phenylalanine (alpha-MF)
  MISC_FEATURE (24)..(24): Xaa is Glutamine, Nle(epsilon-alkyne), or Lysine conjugated via its epsilon amino group to a non-peptide linker comprising a terminal alkyne group
  MISC_FEATURE (25)..(25): Xaa is Tryptophan or alpha-methyl Tryptophan (alpha-MW)
  MISC_FEATURE (26)..(26): Xaa is Leucine or alpha-ML
  MISC_FEATURE (27)..(27): Xaa is methionine, Leucine, methionine sulfoxide, or L-methionine sulphone (2)
  MISC_FEATURE (28)..(28): Xaa is Aspartic acid, Alanine, Lysine, Asparagine, gamma-Glu, Glutamine, or alpha-MD
  MISC_FEATURE (29)..(29): Xaa is Threonine or Glycine
  MISC_FEATURE (30)..(30): Xaa is Arginine, Lysine, or Nle(epsilon-alkyne), or Xaa is absent and
  MISC_FEATURE (31)..(31): Xaa is Glycine, gamma-Glu, Nle(epsilon-alkyne), or Lysine conjugated via its epsilon amino group to a non-peptide linker comprising a terminal alkyne group, or Xaa is absent
XXQGTFTSXXSXYXDXXXAXXFVXXXXXXXX

SEQ ID NO: 10 - protein, 31 aa, Artificial Sequence
  Peptide
  PEPTIDE (1)..(31): C-terminal amino acid optionally is linked to a protecting group or amidated
  PEPTIDE (1)..(31): with the proviso that either X10 is a Lysine residue conjugated to a gamma-Glu-gamma-Glu-C16 and one of X20, X21, X24, X30, or X31 comprises azide or N3 group or X20 is a Lysine residue conjugated to  PEG2PEG2-gamma-Glu-C18-OH or
  PEPTIDE (1)..(31): the PEG2PEG2gamma-E-C20-OH and one of  X21, X24, X30, or X31 comprises the azide or N3 group
  MISC_FEATURE (2)..(2): Xaa is aminoisobutyric acid (Aib), D-Serine (s), or alpha-methyl Serine (alpha-MS)
  MISC_FEATURE (9)..(9): Xaa is Serine or alpha-methyl Aspartic acid (alpha-MD)
  MISC_FEATURE (10)..(10): Xaa is Tyr or Lys conjugated to gamma-Glu-gamma-Glu-C16
  MISC_FEATURE (12)..(12): Xaa is Lysine, Leucine, or Serine
  MISC_FEATURE (14)..(14): Xaa is Leu of alpha-methyl Leucine (alpha-ML)
  MISC_FEATURE (16)..(16): Xaa is Glutamic acid, Asparagine, Serine, Alanine, or Aib
  MISC_FEATURE (17)..(17): Xaa is Arginine or Lysine
  MISC_FEATURE (18)..(18): Xaa is Alanine or Arginine
  MISC_FEATURE (20)..(20): Xaa is Glutamine or Lysine conjugated via its epsilon amine group to PEG2-C5N3, PEG2PEG2-C5N3, PEG2PEG2-gamma-Glu-C16N3, PEG2PEG2-gamma-Glu-C18-OH, or PEG2PEG2gamma-E-C20-OH
  MISC_FEATURE (21)..(21): Xaa is Aspartic acid, alpha-methyl Phenylalanine (alpha-MF), alpha-MD, Azidonorleucine (Norleucine conjugated to an azide group (Nle(epsilon-N3))), or Lys conjugated via its epsilon amine group to PEG2-C5N3 , PEG2PEG2-C5N3, or PEG2PEG2-gamma-Glu-C16N3
  MISC_FEATURE (24)..(24): Xaa is Glutamine, Nle(epsilon-N3), or Lysine conjugated to PEG2PEG2-gamma-Glu-C16N3
  MISC_FEATURE (25)..(25): Xaa is Tryptophan or alpha-methyl Tryptophan (alpha-MW)
  MISC_FEATURE (26)..(26): Xaa is Leucine or alpha-ML
  MISC_FEATURE (27)..(27): Xaa is Leucine or L-methionine sulphone (2)
  MISC_FEATURE (28)..(28): Xaa is Aspartic acid, Alanine, Lysine, Asparagine, gamma-Glu, Glutamine, or alpha-MD
  MISC_FEATURE (29)..(29): Xaa is Threonine or Glycine
  MISC_FEATURE (30)..(30): Xaa is Arginine, Lysine, or Nle(epsilon-N3), or Xaa is absent and
  MISC_FEATURE (31)..(31): Xaa is Glycine, gamma-Glu, Nle(epsilon-N3), or Lysine conjugated via its epsilon amine group to PEG2PEG2-gamma-Glu-C16N3 , PEG2-C5N3 or PEG2PEG2-C5N3, or Xaa is absent
HXQGTFTSXXSXYXDXXXAXXFVXXXXXXXX

SEQ ID NO: 11 - protein, 31 aa, Artificial Sequence; identical to SEQ ID NO: 10
  Peptide
  PEPTIDE (1)..(31): C-terminal amino acid optionally is linked to a protecting group or amidated
  PEPTIDE (1)..(31): with the proviso that either X10 is a Lysine residue conjugated to a gamma-Glu-gamma-Glu-C16 and one of X20, X21, X24, X30, or X31 comprises the -alkyne or X20 is a Lysine residue conjugated to the PEG2PEG2-gamma-Glu-C18-OH or the PEG2PEG2gamma-E-C20-OH
  PEPTIDE (1)..(31): and one of  X21, X24, X30, or X31 comprises the -alkyne
  MISC_FEATURE (2)..(2): Xaa is aminoisobutyric acid (Aib), D-Serine (s), or alpha-methyl Serine (alpha-MS)
  MISC_FEATURE (9)..(9): Xaa is Serine or alpha-methyl Aspartic acid (alpha-MD)
  MISC_FEATURE (10)..(10): Xaa is Tyr or Lys conjugated to gamma-Glu-gamma-Glu-C16
  MISC_FEATURE (12)..(12): Xaa is Lysine, Leucine, or Serine
  MISC_FEATURE (14)..(14): Xaa is Leu of alpha-methyl Leucine (alpha-ML)
  MISC_FEATURE (16)..(16): Xaa is Glutamic acid, Asparagine, Serine, Alanine, or Aib
  MISC_FEATURE (18)..(18): Xaa is Alanine or Arginine
  MISC_FEATURE (20)..(20): X20 is Glutamine or Lysine conjugated via its epsilon amine group to PEG2-C5N3, PEG2PEG2-C5-alkyne, PEG2PEG2-gamma-Glu-C16-alkyne, PEG2PEG2-gamma-Glu-C18-OH, or PEG2PEG2gamma-E-C20-OH
  MISC_FEATURE (21)..(21): Xaa is Aspartic acid, alpha-methyl Phenylalanine (alpha-MF), alpha-MD, Alkynylnorleucine (Norleucine conjugated via its epsilon carbon to an alkyne group (Nle(epsilon-alkyne))), or Lys conjugated v to PEG2-C5-alkyne, PEG2PEG2-C5-alkyne
  MISC_FEATURE (24)..(24): Xaa is Glutamine, Nle(epsilon-alkyne), or Lysine conjugated to PEG2PEG2-gamma-Glu-C16-alkyne
  MISC_FEATURE (25)..(25): Xaa is Tryptophan or alpha-methyl Tryptophan (alpha-MW)
  MISC_FEATURE (26)..(26): Xaa is Leucine or alpha-ML
  MISC_FEATURE (27)..(27): Xaa is Leucine or L-methionine sulphone (2)
  MISC_FEATURE (28)..(28): Xaa is Aspartic acid, Alanine, Lysine, Asparagine, gamma-Glu, Glutamine, or alpha-MD
  MISC_FEATURE (29)..(29): Xaa is Threonine or Glycine
  MISC_FEATURE (30)..(30): Xaa is Arginine, Lysine, or Nle(epsilon-alkyne), or Xaa is absent and
  MISC_FEATURE (31)..(31): Xaa is Glycine, gamma-Glu, Nle(epsilon-alkyne), or Lysine conjugated via its epsilon amine group to PEG2PEG2-gamma-Glu-C16-alkyne, PEG2-C5-alkyne, PEG2PEG2-C5-alkyne, or Xaa is absent

SEQ ID NO: 12 - protein, 31 aa, Artificial Sequence
  Peptide
  PEPTIDE (1)..(31): C-terminal amino acid optionally is linked to a protecting group or amidated
  PEPTIDE (1)..(31): with the proviso that either X10 is a Lysine residue conjugated to a gamma-Glu-gamma-Glu-C16 and one of X20, X21, X24, X30, or X31 comprises the azide or N3 group or X20 is a Lysine residue conjugated to the PEG2PEG2-gamma-Glu-C18-OH or
  PEPTIDE (1)..(31): the PEG2PEG2gamma-E-C20-OH and one of  X21, X24, X30, or X31 comprises the azide or N3 group
  MISC_FEATURE (2)..(2): Xaa is aminoisobutyric acid (Aib), D-Serine (s), or alpha-methyl Serine (alpha-MS)
  MISC_FEATURE (3)..(3): Xaa is Glu or Asp
  MISC_FEATURE (9)..(9): Xaa is Serine or alpha-methyl Aspartic acid (alpha-MD)
  MISC_FEATURE (10)..(10): Xaa is Tyr or Lys conjugated to gamma-Glu-gamma-Glu-C16
  MISC_FEATURE (12)..(12): Xaa is Lysine, Leucine, or Serine
  MISC_FEATURE (14)..(14): Xaa is Leu of alpha-methyl Leucine (alpha-ML)
  MISC_FEATURE (16)..(16): Xaa is Glutamic acid, Asparagine, Serine, Alanine, or Aib
  MISC_FEATURE (17)..(17): Xaa is Arginine or Lysine
  MISC_FEATURE (18)..(18): Xaa is Alanine or Arginine
  MISC_FEATURE (20)..(20): Xaa is Glutamine or Lysine conjugated via its epsilon amine group to PEG2-C5N3, PEG2PEG2-C5N3, PEG2PEG2-gamma-Glu-C16N3, PEG2PEG2-gamma-Glu-C18-OH, or PEG2PEG2gamma-E-C20-OH
  MISC_FEATURE (21)..(21): X21 is Aspartic acid, alpha-methyl Phenylalanine (alpha-MF), alpha-MD, Azidonorleucine (Norleucine conjugated via its epsilon carbon to an azide group (Nle(epsilon-N3))), or Lys conjugated v to PEG2-C5N3 , PEG2PEG2-C5N3, or PEG2PEG2-gamma-Glu-C16N3
  MISC_FEATURE (24)..(24): Xaa is Glutamine, Nle(epsilon-N3), or Lysine conjugated to PEG2PEG2-gamma-Glu-C16N3
  MISC_FEATURE (25)..(25): Xaa is Tryptophan or alpha-methyl Tryptophan (alpha-MW)
  MISC_FEATURE (26)..(26): Xaa is Leucine or alpha-ML
  MISC_FEATURE (27)..(27): Xaa is Leucine or L-methionine sulphone (2)
  MISC_FEATURE (28)..(28): Xaa is Aspartic acid, Alanine, Lysine, Asparagine, gamma-Glu, Glutamine, or alpha-MD
  MISC_FEATURE (30)..(30): Xaa is Arginine, Lysine, or Nle(epsilon-N3), or X30 is absent
  MISC_FEATURE (31)..(31): Xaa is Glycine, gamma-Glu, Nle(epsilon-N3), or Lysine conjugated via its epsilon amine group to PEG2PEG2-gamma-Glu-C16N3 , PEG2-C5N3 or PEG2PEG2-C5N3, or Xaa is absent
HXXGTFTSXXSXYXDXXXAXXFVXXXXXXXX

SEQ ID NO: 13 - protein, 31 aa, Artificial Sequence; identical to SEQ ID NO: 12
  Pepetide
  PEPTIDE (1)..(31): C-terminal amino acid optionally is linked to a protecting group or amidated
  PEPTIDE (1)..(31): with the proviso that either X10 is a Lysine residue conjugated to a gamma-Glu-gamma-Glu-C16 and one of X20, X21, X24, X30, or X31 comprises the -alkyne or X20 is a Lysine residue conjugated to the PEG2PEG2-gamma-Glu-C18-OH or
  PEPTIDE (1)..(31): the PEG2PEG2gamma-E-C20-OH and one of  X21, X24, X30, or X31 comprises the -alkyne
  MISC_FEATURE (2)..(2): Xaa is aminoisobutyric acid (Aib), D-Serine (s), or alpha-methyl Serine (alpha-MS)
  MISC_FEATURE (3)..(3): Xaa is Glu or Asp
  MISC_FEATURE (9)..(9): Xaa is Serine or alpha-methyl Aspartic acid (alpha-MD)
  MISC_FEATURE (10)..(10): Xaa is Tyr or Lys conjugated to gamma-Glu-gamma-Glu-C16
  MISC_FEATURE (12)..(12): Xaa is Lysine, Leucine, or Serine
  MISC_FEATURE (14)..(14): Xaa is Leu of alpha-methyl Leucine (alpha-ML)
  MISC_FEATURE (16)..(16): Xaa is Glutamic acid, Asparagine, Serine, Alanine, or Aib
  MISC_FEATURE (17)..(17): Xaa is Arginine or Lysine
  MISC_FEATURE (18)..(18): Xaa is Alanine or Arginine
  MISC_FEATURE (20)..(20): Xaa is Glutamine or Lysine conjugated via its epsilon amine group to PEG2-C5N3, PEG2PEG2-C5-alkyne, PEG2PEG2-gamma-Glu-C16-alkyne, PEG2PEG2-gamma-Glu-C18-OH, or PEG2PEG2gamma-E-C20-OH
  MISC_FEATURE (21)..(21): Xaa is Aspartic acid, alpha-methyl Phenylalanine (alpha-MF), alpha-MD, Alkynylnorleucine (Norleucine conjugated to an alkyne group (Nle(epsilon-alkyne))), or Lys conjugated  to PEG2-C5-alkyne, PEG2PEG2-C5-alkyne, or
  MISC_FEATURE (24)..(24): Xaa is Glutamine, Nle(epsilon-alkyne), or Lysine conjugated to PEG2PEG2-gamma-Glu-C16-alkyne
  MISC_FEATURE (25)..(25): Xaa is Tryptophan or alpha-methyl Tryptophan (alpha-MW)
  MISC_FEATURE (26)..(26): Xaa is Leucine or alpha-ML
  MISC_FEATURE (27)..(27): Xaa is Leucine or L-methionine sulphone (2)
  MISC_FEATURE (28)..(28): Xaa is Aspartic acid, Alanine, Lysine, Asparagine, gamma-Glu, Glutamine, or alpha-MD
  MISC_FEATURE (29)..(29): Xaa is Threonine or Glycine
  MISC_FEATURE (30)..(30): Xaa is Arginine, Lysine, or Nle(epsilon-alkyne), or Xaa is absent and
  MISC_FEATURE (31)..(31): Xaa is Glycine, gamma-Glu, Nle(epsilon-alkyne), or Lysine conjugated via its epsilon amine group to PEG2PEG2-gamma-Glu-C16-alkyne, PEG2-C5-alkyne, PEG2PEG2-C5-alkyne, or Xaa is absent

SEQ ID NO: 14 - protein, 31 aa, Artificial Sequence
  Peptide
  MISC_FEATURE (1)..(1): Xaa is Tyrosine, Phenylalanine, Tryptophan, or other amino acid with an aromatic group
  PEPTIDE (1)..(31): C-terminal amino acid optionally is linked to a protecting group or amidated
  PEPTIDE (1)..(31): with the proviso that either X10 is a Lysine residue conjugated to a gamma-Glu-gamma-Glu-C16 and one of X20, X21, X24, X30, or X31 comprises the azide or N3 group or X20 is a Lysine residue conjugated to the PEG2PEG2-gamma-Glu-C18-OH or
  PEPTIDE (1)..(31): the PEG2PEG2gamma-E-C20-OH and one of  X21, X24, X30, or X31 comprises the azide or N3 group
  MISC_FEATURE (2)..(2): Xaa is aminoisobutyric acid (Aib), D-Serine (s), or alpha-methyl Serine (alpha-MS)
  MISC_FEATURE (3)..(3): Xaa is Glu or Asp
  MISC_FEATURE (9)..(9): Xaa is Serine or alpha-methyl Aspartic acid (alpha-MD)
  MISC_FEATURE (10)..(10): Xaa is Tyr or Lys conjugated to gamma-Glu-gamma-Glu-C16
  MISC_FEATURE (12)..(12): Xaa is Isoleucine, Lysine, Leucine, or Serine
  MISC_FEATURE (14)..(14): Xaa is Leu of alpha-methyl Leucine (alpha-ML)
  MISC_FEATURE (16)..(16): Xaa is Glutamic acid, Asparagine, Serine, Alanine, or Aib
  MISC_FEATURE (17)..(17): Xaa is Arginine or Lysine
  MISC_FEATURE (18)..(18): Xaa is Alanine or Arginine
  MISC_FEATURE (20)..(20): Xaa is Glutamine or Lysine conjugated via its epsilon amine group to PEG2-C5N3, PEG2PEG2-C5N3, PEG2PEG2-gamma-Glu-C16N3, PEG2PEG2-gamma-Glu-C18-OH, or PEG2PEG2gamma-E-C20-OH
  MISC_FEATURE (21)..(21): Xaa is Aspartic acid, alpha-methyl Phenylalanine (alpha-MF), alpha-MD, Azidonorleucine (Norleucine conjugated via its epsilon carbon to an azide group (Nle(epsilon-N3))), or Lys conjugated to PEG2-C5N3 , PEG2PEG2-C5N3, or PEG2PEG2-gamma-Glu-C16N3
  MISC_FEATURE (24)..(24): Xaa is Glutamine, Nle(epsilon-N3), or Lysine conjugated to PEG2PEG2-gamma-Glu-C16N3
  MISC_FEATURE (25)..(25): Xaa is Tryptophan or alpha-methyl Tryptophan (alpha-MW)
  MISC_FEATURE (26)..(26): Xaa is Leucine or alpha-ML
  MISC_FEATURE (27)..(27): Xaa is Leucine or L-methionine sulphone (2)
  MISC_FEATURE (28)..(28): Xaa is Aspartic acid, Alanine, Lysine, Asparagine, gamma-Glu, Glutamine, or alpha-MD
  MISC_FEATURE (29)..(29): Xaa is Threonine or Glycine
  MISC_FEATURE (30)..(30): Xaa is Arginine, Lysine, or Nle(epsilon-N3), or Xaa is absent
  MISC_FEATURE (31)..(31): Xaa is Glycine, gamma-Glu, Nle(epsilon-N3), or Lysine conjugated via its epsilon amine group to PEG2PEG2-gamma-Glu-C16N3 , PEG2-C5N3 or PEG2PEG2-C5N3, or Xaa is absent
XXXGTFTSXXSXYXDXXXAXXFVXXXXXXXX

SEQ ID NO: 15 - protein, 31 aa, Artificial Sequence; identical to SEQ ID NO: 14
  Peptide
  MISC_FEATURE (1)..(1): Xaa is Tyrosine, Phenylalanine, Tryptophan, or other amino acid with an aromatic group
  PEPTIDE (1)..(31): wherein the C-terminal amino acid optionally is amidated
  PEPTIDE (1)..(31): C-terminal amino acid optionally is linked to a protecting group or amidated
  PEPTIDE (1)..(31): with the proviso that either X10 is a Lysine residue conjugated to a gamma-Glu-gamma-Glu-C16 and one of X20, X21, X24, X30, or X31 comprises the -alkyne or X20 is a Lysine residue conjugated to the PEG2PEG2-gamma-Glu-C18-OH or
  PEPTIDE (1)..(31): the PEG2PEG2gamma-E-C20-OH and one of  X21, X24, X30, or X31 comprises the -alkyne
  MISC_FEATURE (2)..(2): Xaa is aminoisobutyric acid (Aib), D-Serine (s), or alpha-methyl Serine (alpha-MS)
  MISC_FEATURE (3)..(3): Xaa is Glu or Asp
  MISC_FEATURE (9)..(9): Xaa is Serine or alpha-methyl Aspartic acid (alpha-MD)
  MISC_FEATURE (10)..(10): Xaa is Tyr or Lys conjugated to gamma-Glu-gamma-Glu-C16
  MISC_FEATURE (12)..(12): Xaa is Isoleucine, Lysine, Leucine, or Serine
  MISC_FEATURE (14)..(14): Xaa is Leu of alpha-methyl Leucine (alpha-ML)
  MISC_FEATURE (16)..(16): Xaa is Glutamic acid, Asparagine, Serine, Alanine, or Aib
  MISC_FEATURE (17)..(17): Xaa is Arginine or Lysine
  MISC_FEATURE (18)..(18): Xaa is Alanine or Arginine
  MISC_FEATURE (20)..(20): Xaa is Glutamine or Lysine conjugated via its epsilon amine group to PEG2-C5N3, PEG2PEG2-C5-alkyne, PEG2PEG2-gamma-Glu-C16-alkyne, PEG2PEG2-gamma-Glu-C18-OH, or PEG2PEG2gamma-E-C20-OH
  MISC_FEATURE (21)..(21): Xaa is Aspartic acid, alpha-methyl Phenylalanine (alpha-MF), alpha-MD, Alkynylnorleucine (Norleucine conjugated  to an alkyne group (Nle(epsilon-alkyne))), or Lys conjugated to PEG2-C5-alkyne, PEG2PEG2-C5-alkyne, or PEG2PEG2-gamma-Glu-C16
  MISC_FEATURE (24)..(24): Xaa is Glutamine, Nle(epsilon-alkyne), or Lysine conjugated to PEG2PEG2-gamma-Glu-C16-alkyne
  MISC_FEATURE (25)..(25): Xaa is Tryptophan or alpha-methyl Tryptophan (alpha-MW)
  MISC_FEATURE (26)..(26): Xaa is Leucine or alpha-ML
  MISC_FEATURE (27)..(27): Xaa is Leucine or L-methionine sulphone (2)
  MISC_FEATURE (28)..(28): Xaa is Aspartic acid, Alanine, Lysine, Asparagine, gamma-Glu, Glutamine, or alpha-MD
  MISC_FEATURE (29)..(29): Xaa is Threonine or Glycine
  MISC_FEATURE (30)..(30): Xaa is Arginine, Lysine, or Nle(epsilon-alkyne), or Xaa is absent and
  MISC_FEATURE (31)..(31): Xaa is Glycine, gamma-Glu, Nle(epsilon-alkyne), or Lysine conjugated via its epsilon amine group to PEG2PEG2-gamma-Glu-C16-alkyne, PEG2-C5-alkyne, PEG2PEG2-C5-alkyne, or Xaa is absent

SEQ ID NO: 16 - protein, 31 aa, Artificial Sequence; identical to SEQ ID NO: 9
  Peptide
  MISC_FEATURE (1)..(1): Xaa is Tyrosine, Phenylalanine, Tryptophan, or other amino acid with an aromatic group
  PEPTIDE (1)..(31): C-terminal amino acid optionally is linked to a protecting group or amidated
  PEPTIDE (1)..(31): with the proviso that either X10 is a Lysine residue conjugated to a gamma-Glu-gamma-Glu-C16 and one of X20, X21, X24, X30, or X31 comprises the azide or N3 group or X20 is a Lysine residue conjugated to the PEG2PEG2-gamma-Glu-C18-OH or
  PEPTIDE (1)..(31): the PEG2PEG2gamma-E-C20-OH and one of  X21, X24, X30, or X31 comprises the azide or N3 group
  MISC_FEATURE (2)..(2): Xaa is aminoisobutyric acid (Aib), D-Serine (s), or alpha-methyl Serine (alpha-MS)
  MISC_FEATURE (9)..(9): Xaa is Serine or alpha-methyl Aspartic acid (alpha-MD)
  MISC_FEATURE (10)..(10): Xaa is Tyr or Lys conjugated to gamma-Glu-gamma-Glu-C16
  MISC_FEATURE (12)..(12): Xaa is Isoleucine, Lysine, Leucine, or Serine
  MISC_FEATURE (14)..(14): Xaa is Leu of alpha-methyl Leucine (alpha-ML)
  MISC_FEATURE (16)..(16): Xaa is Glutamic acid, Asparagine, Serine, Alanine, or Aib
  MISC_FEATURE (17)..(17): Xaa is Arginine or Lysine
  MISC_FEATURE (18)..(18): Xaa is Alanine or Arginine
  MISC_FEATURE (20)..(20): X20 is Glutamine or Lysine conjugated via its epsilon amine group to PEG2-C5N3, PEG2PEG2-C5N3, PEG2PEG2-gamma-Glu-C16N3, PEG2PEG2-gamma-Glu-C18-OH, or PEG2PEG2gamma-E-C20-OH
  MISC_FEATURE (21)..(21): Xaa is Aspartic acid, alpha-methyl Phenylalanine (alpha-MF), alpha-MD, Azidonorleucine (Norleucine conjugated via its epsilon carbon to an azide group (Nle(epsilon-N3))), or Lys conjugated to PEG2-C5N3 , PEG2PEG2-C5N3, or PEG2PEG2-gamma-Glu-C16N3
  MISC_FEATURE (24)..(24): Xaa is Glutamine, Nle(epsilon-N3), or Lysine conjugated to PEG2PEG2-gamma-Glu-C16N3
  MISC_FEATURE (25)..(25): Xaa is Tryptophan or alpha-methyl Tryptophan (alpha-MW)
  MISC_FEATURE (26)..(26): Xaa is Leucine or alpha-ML
  MISC_FEATURE (27)..(27): Xaa is Leucine or L-methionine sulphone (2)
  MISC_FEATURE (28)..(28): Xaa is Aspartic acid, Alanine, Lysine, Asparagine, gamma-Glu, Glutamine, or alpha-MD
  MISC_FEATURE (29)..(29): Xaa is Threonine or Glycine
  MISC_FEATURE (30)..(30): Xaa is Arginine, Lysine, or Nle(epsilon-N3), or Xaa is absent
  MISC_FEATURE (31)..(31): Xaa is Glycine, gamma-Glu, Nle(epsilon-N3), or Lysine conjugated via its epsilon amine group to PEG2PEG2-gamma-Glu-C16N3 , PEG2-C5N3 or PEG2PEG2-C5N3, or Xaa is absent

SEQ ID NO: 17 - protein, 31 aa, Artificial Sequence; identical to SEQ ID NO: 9
  Peptide
  MISC_FEATURE (1)..(1): Xaa is Tyrosine, Phenylalanine, Tryptophan, or other amino acid with an aromatic group
  PEPETIDE (1)..(31): C-terminal amino acid optionally is linked to a protecting group or amidated
  PEPETIDE (1)..(31): with the proviso that either X10 is a Lysine residue conjugated to a gamma-Glu-gamma-Glu-C16 and one of X20, X21, X24, X30, or X31 comprises the -alkyne or X20 is a Lysine residue conjugated to the PEG2PEG2-gamma-Glu-C18-OH or
  PEPETIDE (1)..(31): the PEG2PEG2gamma-E-C20-OH and one of  X21, X24, X30, or X31
  MISC_FEATURE (2)..(2): Xaa is aminoisobutyric acid (Aib), D-Serine (s), or alpha-methyl Serine (alpha-MS)
  MISC_FEATURE (9)..(9): Xaa is Serine or alpha-methyl Aspartic acid (alpha-MD)
  MISC_FEATURE (10)..(10): Xaa is Tyr or Lys conjugated to gamma-Glu-gamma-Glu-C16
  MISC_FEATURE (12)..(12): Xaa is Isoleucine, Lysine, Leucine, or Serine
  MISC_FEATURE (14)..(14): Xaa is Leu of alpha-methyl Leucine (alpha-ML)
  MISC_FEATURE (16)..(16): Xaa is Glutamic acid, Asparagine, Serine, Alanine, or Aib
  MISC_FEATURE (17)..(17): Xaa is Arginine or Lysine
  MISC_FEATURE (18)..(18): Xaa is Alanine or Arginine
  MISC_FEATURE (20)..(20): Xaa is Glutamine or Lysine conjugated via its epsilon amine group to PEG2-C5N3, PEG2PEG2-C5-alkyne, PEG2PEG2-gamma-Glu-C16-alkyne, PEG2PEG2-gamma-Glu-C18-OH, or PEG2PEG2gamma-E-C20-OH
  MISC_FEATURE (21)..(21): Xaa is Asp, alpha-methyl Phenylalanine (alpha-MF), alpha-MD, Alkynylnorleucine (Norleucine conjugated via its epsilon carbon to an alkyne group (Nle(epsilon-alkyne))), or Lys conjugated to PEG2-C5-alkyne, PEG2PEG2-C5-alkyne, or
  MISC_FEATURE (24)..(24): Xaa is Glutamine, Nle(epsilon-alkyne), or Lysine conjugated to PEG2PEG2-gamma-Glu-C16-alkyne
  MISC_FEATURE (25)..(25): Xaa is Tryptophan or alpha-methyl Tryptophan (alpha-MW)
  MISC_FEATURE (26)..(26): Xaa is Leucine or alpha-ML
  MISC_FEATURE (27)..(27): Xaa is Leucine or L-methionine sulphone (2)
  MISC_FEATURE (28)..(28): Xaa is Aspartic acid, Alanine, Lysine, Asparagine, gamma-Glu, Glutamine, or alpha-MD
  MISC_FEATURE (29)..(29): Xaa is Threonine or Glycine
  MISC_FEATURE (30)..(30): Xaa is Arginine, Lysine, or Nle(epsilon-alkyne), or Xaa is absent
  MISC_FEATURE (31)..(31): X31 is Glycine, gamma-Glu, Nle(epsilon-alkyne), or Lysine conjugated via its epsilon amine group to PEG2PEG2-gamma-Glu-C16-alkyne, PEG2-C5-alkyne, PEG2PEG2-C5-alkyne, or Xaa is absent

SEQ ID NO: 18 - protein, 32 aa, Artificial Sequence
  Peptide
  PEPTIDE (1)..(32): with the proviso that only one of X10, X20, X21, or X28, or X29 is Nle(epsilon-N3) or Lysine conjugated via its epsilon amine group to PEG2PEG2-gamma-Glu-C16- N3, PEG2-C5- N3, PEG2PEG2-C5- N3
  PEPTIDE (1)..(32): C-terminal amino acid optionally is linked to a protecting group or amidated
  MISC_FEATURE (10)..(10): Xaa is Valine, Nle(epsilon-N3), or Lysine conjugated via its epsilon amine group to PEG2PEG2-gamma-Glu-C16- N3, PEG2-C5- N3, or PEG2PEG2-C5- N3
  MISC_FEATURE (20)..(20): Xaa is Lysine, Nle(epsilon-N3), or Lysine conjugated via its epsilon amine group to PEG2PEG2-gamma-Glu-C16- N3, PEG2-C5- N3, or PEG2PEG2-C5- N3
  MISC_FEATURE (21)..(21): Xaa is glutamic acid, Nle(epsilon-N3), or Lysine conjugated via its epsilon amine group to PEG2PEG2-gamma-Glu-C16- N3, PEG2-C5- N3, or PEG2PEG2-C5- N3
  MISC_FEATURE (28)..(28): Xaa is Lysine, Nle(epsilon-N3), or Lysine conjugated via its epsilon amine group to PEG2PEG2-gamma-Glu-C16- N3, PEG2-C5- N3, or PEG2PEG2-C5- N3
  MISC_FEATURE (32)..(32): Xaa Nle(epsilon-N3), or Lysine conjugated via its epsilon amine group to PEG2PEG2-gamma-Glu-C16- N3, PEG2-C5- N3, PEG2PEG2-C5- N3 or absent
HGEGTFTSDXSSYLEEQAAXXFIAWLVXGGGX

SEQ ID NO: 19 - protein, 32 aa, Artificial Sequence; identical to SEQ ID NO: 18
  Peptide
  PEPTIDE (1)..(32): with the proviso that only one of X10, X20, X21, or X28, or X29 is Nle(epsilon-N3) or Lysine conjugated via its epsilon amine group to PEG2PEG2-gamma-Glu-C16-alkyne, PEG2-C5-alkyne, PEG2PEG2-C5-alkyne
  PEPTIDE (1)..(32): C-terminal amino acid optionally is linked to a protecting group or amidated
  MISC_FEATURE (10)..(10): Xaa is Valine, Nle(epsilon-alkyne), or Lysine conjugated via its epsilon amine group to PEG2PEG2-gamma-Glu-C16-alkyne, PEG2-C5-alkyne, or PEG2PEG2-C5-alkyne
  MISC_FEATURE (20)..(20): Xaa is Lysine, Nle(epsilon-N3), or Lysine conjugated via its epsilon amine group to PEG2PEG2-gamma-Glu-C16-alkyne, PEG2-C5-alkyne, or PEG2PEG2-C5-alkyne
  MISC_FEATURE (21)..(21): Xaa is glutamic acid, Nle(epsilon-alkyne), or Lysine conjugated via its epsilon amine group to PEG2PEG2-gamma-Glu-C16-alkyne, PEG2-C5-alkyne, or PEG2PEG2-C5-alkyne
  MISC_FEATURE (28)..(28): Xaa is Lysine, Nle(epsilon-alkyne), or Lysine conjugated via its epsilon amine group to PEG2PEG2-gamma-Glu-C16-alkyne, PEG2-C5-alkyne, or PEG2PEG2-C5-alkyne
  MISC_FEATURE (32)..(32): Xaa Nle(epsilon-alkyne), or Lysine conjugated via its epsilon amine group to PEG2PEG2-gamma-Glu-C16-alkyne, PEG2-C5-alkyne, PEG2PEG2-C5-alkyne or absent

SEQ ID NO: 20 - protein, 29 aa, Artificial Sequence
  Peptide
  MISC_FEATURE (1)..(1): Xaa is His, Phe, or Tyr
  PEPTIDE (1)..(29): C-terminal amino acid optionally is linked to a protecting group or amidated
  PEPTIDE (1)..(29): with provisio that peptide comprises only one Nle(eN3)
  PEPTIDE (1)..(29): optionally the peptide includes a C-terminal extension selected from the group consisting of KK(PEG2PEG2)-C5N3, KQ-Nle(eN3), SEQ ID NO:21, RG-Nle(eN3), SEQ ID NO:22, SEQ ID NO:23, Nle(eN3), KSEQ ID NO:24), and SEQ ID NO:25 linked to the amino acid at 29
  PEPTIDE (1)..(29)
  MISC_FEATURE (2)..(2): Xaa is amionisobutyric acid (Aib), Gly, Ala, Ser, D-Serine (s)
  MISC_FEATURE (3)..(3): Xaa is Glu or Gln
  MISC_FEATURE (7)..(7): Xaa is Tyr
  MISC_FEATURE (9)..(9): Xaa is Asp or Lys
  MISC_FEATURE (10)..(10): Xaa is Tyr, Val, Leu, or Lys
  MISC_FEATURE (11)..(11): Xaa is Ser or Val
  MISC_FEATURE (12)..(12): Xaa is Lysine, Iso, or Serine
  MISC_FEATURE (13)..(13): Xaa is Gln, Ala, or Tyr
  MISC_FEATURE (14)..(14): Xaa is Leu, Met, or met sulphone
  MISC_FEATURE (15)..(15): Xaa is Glu or Asp
  MISC_FEATURE (16)..(16): Xaa is Glu, Asn, Ser, Ala, or Aib
  MISC_FEATURE (17)..(17): Xaa is Glu, Iso, Gln, or Arg
  MISC_FEATURE (18)..(18): Xaa is Ala, His, or Arg
  MISC_FEATURE (19)..(19): Xaa is Val, Gln, or Ala
  MISC_FEATURE (20)..(20): Xaa is Arg, Lys, Gln, or Aib
  MISC_FEATURE (21)..(21): Xaa is Leu, Glu, or Asp
  MISC_FEATURE (23)..(23): Xaa is Iso or Val
  MISC_FEATURE (24)..(24): Xaa is Glu, Ala, Gln, Nle(epsilon-N3), or Lysine conjugated via its epsilon amino group to aPEG2PEG2-gamma-Glu-C16N3
  MISC_FEATURE (27)..(27): Xaa is Lys, Val, Met, Nle(epsilonN3), or Nle
  MISC_FEATURE (28)..(28): Xaa is Asp, Arg, Lys, Ala, or Asn
  MISC_FEATURE (29)..(29): Xaa is Gly, Tyr, Gln, or Gly
XXXGTFXSXXSXYXXXXXXXXFXXWLXXX

SEQ ID NO: 21 - protein, 11 aa, Artificial Sequence
  C-terminal extension
  MISC_FEATURE (11)..(11): Xaa is Nle(epsilon-N3)
GPSSGAPPPSX

SEQ ID NO: 22 - protein, 16 aa, Artificial Sequence
  C-terminal Extension
  MISC_FEATURE (16)..(16): Xaa is Nle(epsilon-N3)
GPSSGAPPSKKKKKKX

SEQ ID NO: 23 - protein, 16 aa, Artificial Sequence
  C-terminal extension
  MISC_FEATURE (16)..(16): Xaa is Nle(epsilon-N3)
GGGGGSGGGSGGGSAX

SEQ ID NO: 24 - protein, 14 aa, Artificial Sequence
  C-terminal extension
  MISC_FEATURE (14)..(14): Xaa is Nle(epsilon-N3)
KGLLNDWKHNITQX

SEQ ID NO: 25 - protein, 9 aa, Artificial Sequence
  C-terminal extension
  MISC_FEATURE (9)..(9): Xaa is Nle(epsilon-N3)
KRNKNNIAX

SEQ ID NO: 26 - protein, 8 aa, Artificial Sequence
  C-terminal extension
KRNKNNIA

SEQ ID NO: 27 - protein, 10 aa, Artificial Sequence
  C-terminal extension
GPSSGAPPPS

SEQ ID NO: 28 - protein, 15 aa, Artificial Sequence
  C-terminal extension
GPSSGAPPSKKKKKK

SEQ ID NO: 29 - protein, 15 aa, Artificial Sequence
  C-terminal extension
GGGGGSGGGSGGGSA

SEQ ID NO: 30 - protein, 13 aa, Artificial Sequence
  C-terminal extension
KGLLNDWKHNITQ

SEQ ID NO: 31 - protein, 29 aa, Artificial Sequence
  Peptide
  MISC_FEATURE (1)..(1): Xaa is His, Phe, or Tyr
  PEPTIDE (1)..(29): wherein the C-terminal amino acid optionally linked to a protecting group or amidated
  PEPTIDE (1)..(29): the peptide includes a C-terminal extension selected from the group consisting of KK(PEG2PEG2)-C5N3, KQ-Nle(eN3), SEQ ID NO:21, RG-Nle(eN3), SEQ ID NO:22, SEQ ID NO:23, Nle(eN3), KSEQ ID NO:24), and SEQ ID NO:25 linked to the amino acid at 29
  PEPTIDE (1)..(29): with proviso peptide comprises only one Nle(eN3)
  MISC_FEATURE (2)..(2): Xaa is amionisobutyric acid (Aib), Gly, Ala, Ser, D-Serine (s)
  MISC_FEATURE (3)..(3): Xaa is Glu or Gln
  MISC_FEATURE (7)..(7): Xaa is Tyr
  MISC_FEATURE (9)..(9): Xaa is Asp or Lys
  MISC_FEATURE (10)..(10): Xaa is Tyr, Val, Leu, or Lys
  MISC_FEATURE (11)..(11): Xaa is Ser or Val
  MISC_FEATURE (12)..(12): Xaa is Lysine, Iso, or Serine
  MISC_FEATURE (13)..(13): Xaa is Gln, Ala, or Tyr
  MISC_FEATURE (14)..(14): Xaa is Leu, Met, or met sulphone
  MISC_FEATURE (15)..(15): Xaa is Glu or Asp
  MISC_FEATURE (16)..(16): Xaa is Glu, Asn, Ser, Ala, or Aib
  MISC_FEATURE (17)..(17): Xaa is Glu, Iso, Gln, or Arg
  MISC_FEATURE (18)..(18): Xaa is Ala, His, or Arg
  MISC_FEATURE (19)..(19): Xaa is Val, Gln, or Ala
  MISC_FEATURE (20)..(20): Xaa is Arg, Lys, Gln, or Aib
  MISC_FEATURE (21)..(21): Xaa is Leu, Glu, or Asp
  MISC_FEATURE (23)..(23): Xaa is Iso or Val
  MISC_FEATURE (24)..(24): Xaa is Glu, Ala, Gln, Nle(epsilon-N3), or Lysine conjugated via its epsilon amino group to aPEG2PEG2-gamma-Glu-C16N3
  MISC_FEATURE (27)..(27): Xaa is Lys, Val, Met, Nle(epsilonN3), or Nle
  MISC_FEATURE (28)..(28): Xaa is Asp, Arg, Lys, Ala, or Asn
  MISC_FEATURE (29)..(29): Xaa is Gly, Tyr, Gln, or Gly
XXXGTFXSXXSXYXXXXXXXXFXXWLXXX

SEQ ID NO: 32-34 - skipped (3 entries)

SEQ ID NO: 35 - protein, 29 aa, Artificial Sequence
  Peptide
  PEPTIDE (1)..(29): C-terminal amide
  MISC_FEATURE (2)..(2): Xaa2 is D-Ser
  MISC_FEATURE (10)..(10): Lys10 conjugated to  gamma-Glu-gamma-Glu-C16
  MISC_FEATURE (21)..(21): Xaa21 is Nle(epsilon-N3)
HXQGTFTSDKSKYLDERAAQXFVQWLLDT

SEQ ID NO: 36 - protein, 31 aa, Artificial Sequence
  Peptide
  PEPTIDE (1)..(31): C-terminal amide
  MISC_FEATURE (2)..(2): Xaa2 is aib
  MISC_FEATURE (10)..(10): Lys10 conjugated to  gamma-Glu-gamma-Glu-C16
  MISC_FEATURE (24)..(24): Xaa24 is Nle(epsilon-N3)
HXQGTFTSDKSKYLDERAAQDFVXWLLDGRG

SEQ ID NO: 37 - protein, 31 aa, Artificial Sequence
  Peptide
  PEPTIDE (1)..(31)
  MISC_FEATURE (2)..(2): Xaa2 is aib
  MISC_FEATURE (10)..(10): Lys10 conjugated to  gamma-Glu-gamma-Glu-C16
  MISC_FEATURE (16)..(16): Xaa16 is aib
  MISC_FEATURE (24)..(24): Xaa24 is Nle(epsilon-N3)
  MISC_FEATURE (27)..(27): Xaa27 is methione sulfone
HXQGTFTSDKSKYLDXRAAQDFVXWLXKGRG

SEQ ID NO: 38 - protein, 31 aa, Artificial Sequence
  Peptide
  PEPTIDE (1)..(31): C-terminal amide
  MISC_FEATURE (2)..(2): Xaa2 is D-Ser
  MISC_FEATURE (10)..(10): Lys10 conjugated to  gamma-Glu-gamma-Glu-C16
  MISC_FEATURE (16)..(16): Xaa16 is aib
  MISC_FEATURE (24)..(24): Xaa24 is Nle(epsilon-N3)
  MISC_FEATURE (31)..(31): Xaa31 is gamma-Glu
HXQGTFTSDKSLYLDXRAAQDFVXWLLNTKX

SEQ ID NO: 39 - protein, 31 aa, Artificial Sequence
  Peptide
  PEPTIDE (1)..(31): C-terminal amide
  MISC_FEATURE (2)..(2): Xaa2 is D-Ser
  MISC_FEATURE (10)..(10): Lys10 conjugated to  gamma-Glu-gamma-Glu-C16
  MISC_FEATURE (16)..(16): Xaa16 is aib
  MISC_FEATURE (30)..(30): Xaa30 is Nle(epsilon-N3)
  MISC_FEATURE (31)..(31): Xaa31 is  gamma-Glu
HXQGTFTSDKSLYLDXRAAQDFVQWLLNTXX

SEQ ID NO: 40 - protein, 31 aa, Artificial Sequence
  Peptide
  PEPTIDE (1)..(31): C-terminal amide
  MISC_FEATURE (2)..(2): Xaa2 is aib
  MISC_FEATURE (10)..(10): Lys10 conjugated to  gamma-Glu-gamma-Glu-C16
  MISC_FEATURE (16)..(16): Xaa16 is aib
  MISC_FEATURE (30)..(30): Xaa30 is Nle(epsilon-N3)
  MISC_FEATURE (31)..(31): Xaa31 is  gamma-Glu
HXQGTFTSDKSKYLDXRRAQDFVQWLLDTXX

SEQ ID NO: 41 - protein, 29 aa, Artificial Sequence
  Peptide
  PEPTIDE (1)..(29): C-terminal amide
  MISC_FEATURE (2)..(2): Xaa2 is D-Ser
  MISC_FEATURE (10)..(10): Lys10 conjugated to  gamma-Glu-gamma-Glu-C16
  MISC_FEATURE (16)..(16): Xaa16 is aib
  MISC_FEATURE (24)..(24): Xaa24 is Nle(epsilon-N3)
HXQGTFTSDKSKYLDXRAAQDFVXWLLDT

SEQ ID NO: 42 - protein, 31 aa, Artificial Sequence
  Peptide
  PEPTIDE (1)..(31): C-terminal amide
  MISC_FEATURE (2)..(2): Xaa2 is D-Ser
  MISC_FEATURE (10)..(10): Lys10 conjugated to  gamma-Glu-gamma-Glu-C16
  MISC_FEATURE (16)..(16): Xaa16 is aib
  MISC_FEATURE (30)..(30): Xaa30 is Nle(epsilon-N3)
  MISC_FEATURE (31)..(31): Xaa31 is  gamma-Glu
HXQGTFTSDKSSYLDXRAAQDFVQWLLNTXX

SEQ ID NO: 43 - protein, 31 aa, Artificial Sequence
  Peptide
  PEPTIDE (1)..(31): C-terminal amide
  MISC_FEATURE (2)..(2): Xaa2 is D-Ser
  MISC_FEATURE (10)..(10): Lys10 conjugated to  gamma-Glu-gamma-Glu-C16
  MISC_FEATURE (16)..(16): Xaa16 is aib
  MISC_FEATURE (24)..(24): Xaa24 is Nle(epsilon-N3)
HXQGTFTSDKSSYLDXRAAQDFVXWLLNTKX

SEQ ID NO: 44 - protein, 29 aa, Artificial Sequence
  Peptide
  PEPTIDE (1)..(29): C-terminal amide
  MISC_FEATURE (2)..(2): Xaa2 is aib
  MISC_FEATURE (10)..(10): Lys10 conjugated to  gamma-Glu-gamma-Glu-C16
  MISC_FEATURE (16)..(16): Xaa16 is aib
  MISC_FEATURE (24)..(24): Xaa24 is Nle(epsilon-N3)
  MISC_FEATURE (27)..(27): Xaa27 is methione sulfone
HXQGTFTSDKSKYLDXRAAQDFVXWLXDT

SEQ ID NO: 45 - protein, 29 aa, Artificial Sequence
  Peptide
  PEPTIDE (1)..(29): C-terminal amide
  MISC_FEATURE (2)..(2): Xaa2 is D-Ser
  MISC_FEATURE (10)..(10): Lys10 conjugated to  gamma-Glu-gamma-Glu-C16
  MISC_FEATURE (24)..(24): Xaa24 is Nle(epsilon-N3)
HXQGTFTSDKSKYLDERAAQDFVXWLLXT

SEQ ID NO: 46 - protein, 29 aa, Artificial Sequence
  Peptide
  PEPTIDE (1)..(29): C-terminal amide
  MISC_FEATURE (2)..(2): Xaa2 is D-Ser
  MISC_FEATURE (10)..(10): Lys10 conjugated to  gamma-Glu-gamma-Glu-C16
  MISC_FEATURE (24)..(24): Xaa24 is Nle(epsilon-N3)
HXQGTFTSDKSKYLDNKRAQDFVXWLLQT

SEQ ID NO: 47 - protein, 29 aa, Artificial Sequence
  Peptide
  PEPTIDE (1)..(29): C-terminal amide
  MISC_FEATURE (2)..(2): Xaa2 is D-Ser
  MISC_FEATURE (10)..(10): Lys10 conjugated to  gamma-Glu-gamma-Glu-C16
  MISC_FEATURE (24)..(24): Xaa24 is Nle(epsilon-N3)
HXQGTFTSDKSKYLDSRRAHDFVXWLLNT

SEQ ID NO: 48 - protein, 29 aa, Artificial Sequence
  Peptide
  PEPTIDE (1)..(29): C-terminal amide
  MISC_FEATURE (2)..(2): Xaa2 is D-Ser
  MISC_FEATURE (10)..(10): Lys10 conjugated to  gamma-Glu-gamma-Glu-C16
  MISC_FEATURE (24)..(24): Lys24 is conjugated to  PEG2-C5N3
HXQGTFTSDKSKYLDERAAQDFVKWLLDT

SEQ ID NO: 49 - protein, 29 aa, Artificial Sequence
  Peptide
  PEPTIDE (1)..(29): C-terminal amide
  MISC_FEATURE (2)..(2): Xaa2 is D-Ser
  MISC_FEATURE (10)..(10): Lys10 conjugated to  gamma-Glu-gamma-Glu-C16
  MISC_FEATURE (24)..(24): Lys24 is conjugated to  PEG2PEG2-C5N3
HXQGTFTSDKSKYLDERAAQDFVKWLLDT

SEQ ID NO: 50 - protein, 29 aa, Artificial Sequence
  Peptide
  PEPTIDE (1)..(29): C-terminal amide
  MISC_FEATURE (2)..(2): Xaa2 is D-Ser
  MISC_FEATURE (10)..(10): Lys10 conjugated to  gamma-Glu-gamma-Glu-C16
  MISC_FEATURE (20)..(20): Lys20 is conjugated to  PEG2-C5N3
HXQGTFTSDKSKYLDERAAKDFVQWLLDT

SEQ ID NO: 51 - protein, 29 aa, Artificial Sequence
  Peptide
  PEPTIDE (1)..(29): C-terminal amide
  MISC_FEATURE (2)..(2): Xaa2 is D-Ser
  MISC_FEATURE (10)..(10): Lys10 conjugated to  gamma-Glu-gamma-Glu-C16
  MISC_FEATURE (20)..(20): Lys20 is conjugated to  PEG2PEG2-C5N3
HXQGTFTSDKSKYLDERAAKDFVQWLLDT

SEQ ID NO: 52 - protein, 31 aa, Artificial Sequence
  Peptide
  PEPTIDE (1)..(31): C-terminal amide
  MISC_FEATURE (2)..(2): Xaa2 is aib
  MISC_FEATURE (16)..(16): Xaa16 is aib
  MISC_FEATURE (31)..(31): Xaa31 is Nle(epsilon-N3)
HXQGTFTSDYSKYLDXRAAQDFVQWLLDTKX

SEQ ID NO: 53 - protein, 31 aa, Artificial Sequence
  Peptide
  PEPTIDE (1)..(31): C-terminal amide
  MISC_FEATURE (2)..(2): Xaa2 is aib
  MISC_FEATURE (10)..(10): Lys10 conjugated to  gamma-Glu-gamma-Glu-C16
  MISC_FEATURE (16)..(16): Xaa16 is aib
  MISC_FEATURE (31)..(31): Xaa31 is Nle(epsilon-N3)
HXQGTFTSDKSKYLDXRAAQDFVQWLLDTKX

SEQ ID NO: 54 - protein, 31 aa, Artificial Sequence
  Peptide
  PEPTIDE (1)..(31): C-terminal amide
  MISC_FEATURE (2)..(2): Xaa2 is aib
  MISC_FEATURE (10)..(10): Lys10 conjugated to  gamma-Glu-gamma-Glu-C16
  MISC_FEATURE (16)..(16): Xaa16 is aib
  MISC_FEATURE (31)..(31): K31 conjugated to  PEG2-C5N3
HXQGTFTSDKSKYLDXRAAQDFVQWLLDTKK

SEQ ID NO: 55 - protein, 31 aa, Artificial Sequence; identical to SEQ ID NO: 54
  Peptide
  PEPTIDE (1)..(31): C-terminal amide
  MISC_FEATURE (2)..(2): Xaa2 is aib
  MISC_FEATURE (10)..(10): Lys10 conjugated to  gamma-Glu-gamma-Glu-C16
  MISC_FEATURE (16)..(16): Xaa16 is aib
  MISC_FEATURE (31)..(31): Lys31 is conjugated to  PEG2PEG2-C5N3

SEQ ID NO: 56 - protein, 31 aa, Artificial Sequence
  Peptide
  PEPTIDE (1)..(31): C-terminal amide
  MISC_FEATURE (2)..(2): Xaa2 is aib
  MISC_FEATURE (10)..(10): Lys10 conjugated to  gamma-Glu-gamma-Glu-C16
  MISC_FEATURE (16)..(16): Xaa16 is aib
  MISC_FEATURE (24)..(24): Xaa24 is Nle(epsilon-N3)
  MISC_FEATURE (31)..(31): X31 is gamma-Glu
HXQGTFTSDKSKYLDXRAAQDFVXWLLDTKX

SEQ ID NO: 57 - protein, 29 aa, Artificial Sequence
  Peptide
  PEPTIDE (1)..(29): C-terminal amide
  MISC_FEATURE (2)..(2): Xaa2 is D-Ser
  MISC_FEATURE (10)..(10): Lys10 conjugated to  gamma-Glu-gamma-Glu-C16
  MISC_FEATURE (21)..(21): Xaa21 is Nle(epsilon-N3)
  MISC_FEATURE (27)..(27): Xaa27 is methione sulfone
HXQGTFTSDKSKYLDERAAQXFVQWLXDT

SEQ ID NO: 58 - protein, 29 aa, Artificial Sequence
  Peptide
  PEPTIDE (1)..(29): C-terminal amide
  MISC_FEATURE (2)..(2): Xaa2 is D-Ser
  MISC_FEATURE (10)..(10): Lys10 conjugated to  gamma-Glu-gamma-Glu-C16
  MISC_FEATURE (21)..(21): Xaa21 is Nle(epsilon-N3)
  MISC_FEATURE (27)..(27): Xaa27 is methione sulfone
  MISC_FEATURE (28)..(28): Xaa28 is alpha-MD
HXQGTFTSDKSKYLDERAAQXFVQWLXXT

SEQ ID NO: 59 - protein, 29 aa, Artificial Sequence
  Peptide
  PEPTIDE (1)..(29): C-terminal amide
  MISC_FEATURE (2)..(2): Xaa2 is D-Ser
  MISC_FEATURE (21)..(21): Xaa21 is Nle(epsilon-N3)
  MISC_FEATURE (24)..(24): Lys24 is conjugated to  PEG2PEG2-gamma-Glu-C16N3
HXQGTFTSDYSKYLDERAAQDFVKWLLDT

SEQ ID NO: 60 - protein, 29 aa, Artificial Sequence
  Peptide
  PEPTIDE (1)..(29): C-terminal amide
  MISC_FEATURE (2)..(2): Xaa2 is D-Ser
  MISC_FEATURE (20)..(20): Lys20 is conjugated to  PEG2PEG2-gamma-Glu-C16N3
HXQGTFTSDYSKYLDERAAKDFVQWLLDT

SEQ ID NO: 61 - protein, 29 aa, Artificial Sequence
  Peptide
  PEPTIDE (1)..(29): C-terminal amide
  MISC_FEATURE (2)..(2): Xaa2 is D-Ser
  MISC_FEATURE (21)..(21): Lys21 is conjugated to  PEG2PEG2gamma-Glu-C16N3
HXQGTFTSDYSKYLDERAAQKFVQWLLDT

SEQ ID NO: 62 - protein, 31 aa, Artificial Sequence
  Peptide
  PEPTIDE (1)..(31): C-terminal amide
  MISC_FEATURE (2)..(2): Xaa2 is aib
  MISC_FEATURE (16)..(16): Xaa16 is aib
  MISC_FEATURE (31)..(31): Lys31 is conjugated to  PEG2PEG2-gamma-Glu-C16N3
HXQGTFTSDYSKYLDXRAAQDFVQWLLDTKK

SEQ ID NO: 63 - protein, 29 aa, Artificial Sequence
  Peptide
  PEPTIDE (1)..(29): C-terminal amide
  MISC_FEATURE (2)..(2): Xaa2 is D-Ser
  MISC_FEATURE (10)..(10): Lys10 is conjugated to  PEG2PEG2-gamma-Glu-C18OH
  MISC_FEATURE (24)..(24): Xaa24 is Nle(epsilon-N3)
HXQGTFTSDKSKYLDERAAQDFVXWLLDT

SEQ ID NO: 64 - protein, 29 aa, Artificial Sequence
  Peptide
  PEPTIDE (1)..(29): C-terminal amide
  MISC_FEATURE (2)..(2): Xaa2 is aib
  MISC_FEATURE (20)..(20): Lys20 is cojugated to  PEG2PEG2-gamma-Glu-C18-OH
  MISC_FEATURE (24)..(24): Xaa24 is Nle(epsilon-N3)
  MISC_FEATURE (27)..(27): Xaa27 is methione sulfone
HXQGTFTSDYSKYLDARAAKDFVXWLXDT

SEQ ID NO: 65 - protein, 29 aa, Artificial Sequence
  Peptide
  PEPTIDE (1)..(29): C-terminal amide
  MISC_FEATURE (2)..(2): Xaa2 is aib
  MISC_FEATURE (20)..(20): Lys20 is conjugated to  PEG2PEG2-gamma-Glu-C20-OH
  MISC_FEATURE (24)..(24): Xaa24 is Nle(epsilon-N3)
  MISC_FEATURE (27)..(27): Xaa27 is methione sulfone
HXQGTFTSDYSKYLDARAAKDFVXWLXDT

SEQ ID NO: 66 - protein, 29 aa, Artificial Sequence
  Peptide
  PEPTIDE (1)..(29): C-terminal amide
  MISC_FEATURE (2)..(2): Xaa2 is D-Ser
  MISC_FEATURE (9)..(9): Xaa9 is alpha-MD
  MISC_FEATURE (10)..(10): Lys10 conjugated to  gamma-Glu-gamma-Glu-C16
  MISC_FEATURE (24)..(24): Xaa24 is Nle(epsilon-N3)
  MISC_FEATURE (27)..(27): Xaa27 is methione sulfone
HXQGTFTSXKSKYLDERAAQDFVXWLXDT

SEQ ID NO: 67 - protein, 29 aa, Artificial Sequence
  Peptide
  PEPTIDE (1)..(29): C-terminal amide
  MISC_FEATURE (2)..(2): Xaa2 is D-Ser
  MISC_FEATURE (10)..(10): Lys10 conjugated to  gamma-Glu-gamma-Glu-C16
  MISC_FEATURE (14)..(14): Xaa14 is alpha-ML
  MISC_FEATURE (24)..(24): Xaa24 is Nle(epsilon-N3)
  MISC_FEATURE (27)..(27): Xaa27 is methione sulfone
HXQGTFTSDKSKYXDERAAQDFVXWLXDT

SEQ ID NO: 68 - protein, 29 aa, Artificial Sequence
  Peptide
  PEPTIDE (1)..(29): C-terminal amide
  MISC_FEATURE (2)..(2): Xaa2 is D-Ser
  MISC_FEATURE (10)..(10): Lys10 conjugated to  gamma-Glu-gamma-Glu-C16
  MISC_FEATURE (21)..(21): Xaa21 is alpha-MD
  MISC_FEATURE (24)..(24): Xaa24 is Nle(epsilon-N3)
  MISC_FEATURE (27)..(27): Xaa27 is methione sulfone
HXQGTFTSDKSKYLDERAAQXFVXWLXDT

SEQ ID NO: 69 - protein, 29 aa, Artificial Sequence
  Peptide
  PEPTIDE (1)..(29): C-terminal amide
  MISC_FEATURE (2)..(2): Xaa2 is D-Ser
  MISC_FEATURE (9)..(9): Xaa9 is alpha-MF
  MISC_FEATURE (10)..(10): Lys10 conjugated to  gamma-Glu-gamma-Glu-C16
  MISC_FEATURE (24)..(24): Xaa24 is Nle(epsilon-N3)
  MISC_FEATURE (27)..(27): Xaa27 is methione sulfone
HXQGTFTSDKSKYLDERAAQDXVXWLXDT

SEQ ID NO: 70 - protein, 29 aa, Artificial Sequence
  Peptide
  PEPTIDE (1)..(29): C-terminal amide
  MISC_FEATURE (2)..(2): Xaa2 is D-Ser
  MISC_FEATURE (10)..(10): Lys10 conjugated to  gamma-Glu-gamma-Glu-C16
  MISC_FEATURE (24)..(24): Xaa24 is Nle(epsilon-N3)
  MISC_FEATURE (25)..(25): Xaa25 is alpha-MW
  MISC_FEATURE (27)..(27): Xaa27 is methione sulfone
HXQGTFTSDKSKYLDERAAQDFVXXLXDT

SEQ ID NO: 71 - protein, 29 aa, Artificial Sequence
  Peptide
  PEPTIDE (1)..(29): C-terminal amide
  MISC_FEATURE (2)..(2): Xaa2 is D-Ser
  MISC_FEATURE (10)..(10): Lys10 conjugated to  gamma-Glu-gamma-Glu-C16
  MISC_FEATURE (24)..(24): Xaa24 is Nle(epsilon-N3)
  MISC_FEATURE (26)..(26): Xaa26 is alpha-ML
  MISC_FEATURE (27)..(27): Xaa27 is methione sulfone
HXQGTFTSDKSKYLDERAAQDFVXWXXDT

SEQ ID NO: 72 - protein, 29 aa, Artificial Sequence
  Peptide
  PEPTIDE (1)..(29): C-terminal amide
  MISC_FEATURE (2)..(2): Xaa2 is D-Ser
  MISC_FEATURE (10)..(10): Lys10 conjugated to  gamma-Glu-gamma-Glu-C16
  MISC_FEATURE (24)..(24): Xaa24 is Nle(epsilon-N3)
  MISC_FEATURE (27)..(27): Xaa27 is methione sulfone
  MISC_FEATURE (28)..(28): Xaa28 is alpha-MD
HXQGTFTSDKSKYLDERAAQDFVXWLXXT

SEQ ID NO: 73 - protein, 31 aa, Artificial Sequence
  Peptide
  PEPTIDE (1)..(31): C-terminal amide
  MISC_FEATURE (2)..(2): Xaa2 is alpha-MS
  MISC_FEATURE (10)..(10): Lys10 conjugated to  gamma-Glu-gamma-Glu-C16
  MISC_FEATURE (16)..(16): Xaa16 is aib
  MISC_FEATURE (24)..(24): Xaa24 is Nle(epsilon-N3)
  MISC_FEATURE (31)..(31): Xaa31 is gamma-Glu
HXQGTFTSDKSKYLDXRAAQDFVXWLLATKX

SEQ ID NO: 74 - protein, 31 aa, Artificial Sequence; identical to SEQ ID NO: 73
  Peptide
  PEPTIDE (1)..(31): C-terminal amide
  MISC_FEATURE (2)..(2): Xaa2 is alpha-Ms
  MISC_FEATURE (10)..(10): Lys10 conjugated to  gamma-Glu-gamma-Glu-C16
  MISC_FEATURE (16)..(16): Xaa16 is aib
  MISC_FEATURE (24)..(24): Xaa24 is Nle(epsilon-N3)
  MISC_FEATURE (31)..(31): Xaa31 is gamma-Glu

SEQ ID NO: 75 - protein, 29 aa, Artificial Sequence
  Peptide
  PEPTIDE (1)..(29): C-terminal amide
  MISC_FEATURE (2)..(2): Xaa2 is alpha-MS
  MISC_FEATURE (10)..(10): Lys10 conjugated to  gamma-Glu-gamma-Glu-C16
  MISC_FEATURE (24)..(24): Xaa24 is Nle(epsilon-N3)
HXQGTFTSDKSKYLDARAAQDFVXWLLDT

SEQ ID NO: 76 - protein, 29 aa, Artificial Sequence
  Peptide
  PEPTIDE (1)..(29): C-terminal amide
  MISC_FEATURE (2)..(2): Xaa2 is alpha-Ms
  MISC_FEATURE (10)..(10): Lys10 conjugated to  gamma-Glu-gamma-Glu-C16
  MISC_FEATURE (24)..(24): Xaa24 is Nle(epsilon-N3)
HXQGTFTSDKSKYLDARAAQDFVXWLLDT

SEQ ID NO: 77 - protein, 29 aa, Artificial Sequence
  Peptide
  PEPTIDE (1)..(29): C-terminal amide
  MISC_FEATURE (2)..(2): Xaa2 is alpha-Ms
  MISC_FEATURE (10)..(10): Lys10 conjugated to  gamma-Glu-gamma-Glu-C16
  MISC_FEATURE (16)..(16): Xaa16 is aib
  MISC_FEATURE (24)..(24): Xaa24 is Nle(epsilon-N3)
  MISC_FEATURE (27)..(27): Xaa27 is methione sulfone
HXVGTFTSDKSKYLDXRAAQDFVXWLXDT

SEQ ID NO: 78 - protein, 31 aa, Artificial Sequence
  Peptide
  PEPTIDE (1)..(31): C-terminal amide
  MISC_FEATURE (2)..(2): Xaa2 is aib
  MISC_FEATURE (10)..(10): Lys10 conjugated to  gamma-Glu-gamma-Glu-C16
  MISC_FEATURE (24)..(24): Xaa24 is Nle(epsilon-N3)
  MISC_FEATURE (27)..(27): Xaa27 is methione sulfone
HXQGTFTSDKSKYLDERAAQDFVXWLXDGRG

SEQ ID NO: 79 - protein, 31 aa, Artificial Sequence
  Peptide
  PEPTIDE (1)..(31): C-terminal amide
  MISC_FEATURE (2)..(2): Xaa2 is aib
  MISC_FEATURE (10)..(10): Lys10 conjugated to  gamma-Glu-gamma-Glu-C16
  MISC_FEATURE (24)..(24): Xaa24 is Nle(epsilon-N3)
  MISC_FEATURE (27)..(27): Xaa27 is methione sulfone
  MISC_FEATURE (28)..(28): Xaa28 is alpha-MD
HXQGTFTSDKSKYLDERAAQDFVXWLXXGRG

SEQ ID NO: 80 - protein, 31 aa, Artificial Sequence
  Peptide
  PEPTIDE (1)..(31): C-terminal amide
  MISC_FEATURE (2)..(2): Xaa2 is aib
  MISC_FEATURE (10)..(10): Lys10 conjugated to  gamma-Glu-gamma-Glu-C16
  MISC_FEATURE (16)..(16): Xaa16 is aib
  MISC_FEATURE (30)..(30): Xaa30 is Nle(epsilon-N3)
  MISC_FEATURE (31)..(31): Xaa31 is  gamma-Glu
HXQGTFTSDKSKYLDXRAAQDFVQWLLDTXX

SEQ ID NO: 81 - protein, 31 aa, Artificial Sequence
  Peptide
  PEPTIDE (1)..(31): C-terminal amide
  MISC_FEATURE (2)..(2): Xaa2 is aib
  MISC_FEATURE (10)..(10): Lys10 conjugated to  gamma-Glu-gamma-Glu-C16
  MISC_FEATURE (16)..(16): Xaa16 is aib
  MISC_FEATURE (27)..(27): Xaa27 is methione sulfone
  MISC_FEATURE (30)..(30): Xaa30 is Nle(epsilon-N3)
  MISC_FEATURE (31)..(31): Xaa31 is  gamma-Glu
HXQGTFTSDKSKYLDXRAAQDFVQWLXDTXX

SEQ ID NO: 82 - protein, 31 aa, Artificial Sequence
  Peptide
  PEPTIDE (1)..(31): C-terminal amide
  MISC_FEATURE (2)..(2): Xaa2 is aib
  MISC_FEATURE (10)..(10): Lys10 conjugated to  gamma-Glu-gamma-Glu-C16
  MISC_FEATURE (16)..(16): Xaa16 is aib
  MISC_FEATURE (27)..(27): Xaa27 is methione sulfone
  MISC_FEATURE (28)..(28): Xaa28 is alpha-MD
  MISC_FEATURE (30)..(30): Xaa30 is Nle(epsilon-N3)
  MISC_FEATURE (31)..(31): Xaa31 is  gamma-Glu
HXQGTFTSDKSKYLDXRAAQDFVQWLXXTXX

SEQ ID NO: 83 - protein, 29 aa, Artificial Sequence
  Peptide
  PEPTIDE (1)..(28)
  MISC_FEATURE (2)..(2): Xaa2 is aib
  MISC_FEATURE (10)..(10): Lys10 conjugated to  gamma-Glu-gamma-Glu-C16
  MISC_FEATURE (16)..(16): Xaa16 is aib
  MISC_FEATURE (24)..(24): Xaa24 is Nle(epsilon-N3)
  MISC_FEATURE (27)..(27): Xaa27 is methione sulfone
  MISC_FEATURE (28)..(28): Xaa28 is alpha-MD
HXQGTFTSDKSKYLDXRAAQDFVXWLXXT

SEQ ID NO: 84 - protein, 29 aa, Artificial Sequence
  Peptide
  PEPTIDE (1)..(29): C-terminal amide
  MISC_FEATURE (2)..(2): Xaa2 is D-Ser
  MISC_FEATURE (10)..(10): Lys10 conjugated to  gamma-Glu-gamma-Glu-C16
  MISC_FEATURE (24)..(24): Xaa24 is Nle(epsilon-N3)
HXEGTFTSDKSKYLDERAAQDFVXWLLDT

SEQ ID NO: 85 - protein, 29 aa, Artificial Sequence
  Peptide
  PEPTIDE (1)..(29): C-terminal amide
  MISC_FEATURE (2)..(2): Xaa2 is D-Ser
  MISC_FEATURE (10)..(10): Lys10 conjugated to  gamma-Glu-gamma-Glu-C16
  MISC_FEATURE (24)..(24): Lys24 is conjugated to  PEG2PEG2-C5N3
  MISC_FEATURE (27)..(27): Xaa27 is methione sulfone
HXQGTFTSDKSKYLDERAAQDFVKWLXDT

SEQ ID NO: 86 - protein, 29 aa, Artificial Sequence
  Peptide
  PEPTIDE (1)..(29): C-terminal amide
  MISC_FEATURE (2)..(2): Xaa2 is D-Ser
  MISC_FEATURE (10)..(10): Lys10 conjugated to  gamma-Glu-gamma-Glu-C16
  MISC_FEATURE (24)..(24): Lys24 is conjugated to  PEG2PEG2-C5N3
  MISC_FEATURE (27)..(27): Xaa27 is methione sulfone
  MISC_FEATURE (28)..(28): Xaa28 is alpha-MD
HXQGTFTSDKSKYLDERAAQDFVKWLXXT

SEQ ID NO: 87 - protein, 29 aa, Artificial Sequence
  Peptide
  PEPTIDE (1)..(29): C-terminal amide
  MISC_FEATURE (2)..(2): Xaa2 is D-Ser
  MISC_FEATURE (10)..(10): Lys10 conjugated to  gamma-Glu-gamma-Glu-C16
  MISC_FEATURE (24)..(24): Lys24 is conjugated to  PEG2-C10N3
HXQGTFTSDKSKYLDERAAQDFVKWLLDT

SEQ ID NO: 88 - protein, 29 aa, Artificial Sequence
  Peptide
  PEPTIDE (1)..(29): C-terminal amide
  MISC_FEATURE (2)..(2): Xaa2 is D-Ser
  MISC_FEATURE (10)..(10): Lys10 conjugated to  gamma-Glu-gamma-Glu-C16
  MISC_FEATURE (24)..(24): Lys24 is conjugated to  PEG2-C16N3
HXQGTFTSDKSKYLDERAAQDFVKWLLDT

SEQ ID NO: 89 - protein, 29 aa, Artificial Sequence
  Peptide
  PEPTIDE (1)..(29): C-terminal amide
  MISC_FEATURE (2)..(2): Xaa2 is aib
  MISC_FEATURE (10)..(10): Lys10 conjugated to  gamma-Glu-gamma-Glu-C16
  MISC_FEATURE (16)..(16): Xaa16 is aib
  MISC_FEATURE (24)..(24): Lys24 is conjugated to PEG2PEG2- C5N3
  MISC_FEATURE (27)..(27): Xaa27 is methione sulfone
HXQGTFTSDKSKYLDXRAAQDFVKWLXDT

SEQ ID NO: 90 - protein, 29 aa, Artificial Sequence
  Peptide
  PEPTIDE (1)..(29): C-terminal amide
  MISC_FEATURE (2)..(2): Xaa2 is aib
  MISC_FEATURE (10)..(10): Lys10 conjugated to  gamma-Glu-gamma-Glu-C16
  MISC_FEATURE (16)..(16): Xaa16 is aib
  MISC_FEATURE (24)..(24): Lys24 is conjugated to PEG2PEG2- C5N3
  MISC_FEATURE (27)..(27): Xaa27 is methione sulfone
HXQGTFTSDKSKYLDXRAAQDFVKWLXDT

SEQ ID NO: 91 - protein, 29 aa, Artificial Sequence
  Peptide
  PEPTIDE (1)..(29): C-terminal amide
  MISC_FEATURE (2)..(2): Xaa2 is D-Ser
  MISC_FEATURE (10)..(10): Lys10 conjugated to  gamma-Glu-gamma-Glu-C16
  MISC_FEATURE (20)..(20): Lys20 is conjugated to PEG2PEG2-gamma-Glu-C10N3
HXQGTFTSDKSKYLDERAAKDFVQWLLDT

SEQ ID NO: 92 - protein, 29 aa, Artificial Sequence
  Peptide
  PEPTIDE (1)..(29): C-terminal amide
  MISC_FEATURE (2)..(2): Xaa2 is D-Ser
  MISC_FEATURE (10)..(10): Lys10 conjugated to  gamma-Glu-gamma-Glu-C16
  MISC_FEATURE (20)..(20): Lys20 is conjugated to PEG2PEG2-gamma-Glu-C16N3
HXQGTFTSDKSKYLDERAAKDFVQWLLDT

SEQ ID NO: 93 - protein, 31 aa, Artificial Sequence; identical to SEQ ID NO: 53
  Peptide
  PEPTIDE (1)..(31): C-terminal amide
  MISC_FEATURE (2)..(2): Xaa2 is D-Ser
  MISC_FEATURE (10)..(10): Lys10 conjugated to  gamma-Glu-gamma-Glu-C16
  MISC_FEATURE (16)..(16): Xaa16 is aib
  MISC_FEATURE (30)..(30): Xaa30 is Nle(epsilon-N3)
  MISC_FEATURE (31)..(31): Xaa31 is  gamma-Glu

SEQ ID NO: 94 - protein, 31 aa, Artificial Sequence
  Peptide
  PEPTIDE (1)..(31): C-terminal amide
  MISC_FEATURE (2)..(2): Xaa2 is D-Ser
  MISC_FEATURE (10)..(10): Lys10 conjugated to  gamma-Glu-gamma-Glu-C16
  MISC_FEATURE (30)..(30): Xaa30 is Nle(epsilon-N3)
  MISC_FEATURE (31)..(31): Xaa31 is  gamma-Glu
HXQGTFTSDKSKYLDERAAQDFVQWLLDTKX

SEQ ID NO: 95 - protein, 31 aa, Artificial Sequence; identical to SEQ ID NO: 54
  Peptide
  PEPTIDE (1)..(31): C-terminal amide
  MISC_FEATURE (2)..(2): Xaa2 is D-Ser
  MISC_FEATURE (10)..(10): Lys10 conjugated to  gamma-Glu-gamma-Glu-C16
  MISC_FEATURE (16)..(16): Xaa16 is aib
  MISC_FEATURE (31)..(31): Xaa31 is conjugated to  PEG2PEG2-C5N3

SEQ ID NO: 96 - protein, 31 aa, Artificial Sequence
  Peptide
  PEPTIDE (1)..(31): C-terminal amide
  MISC_FEATURE (2)..(2): Xaa2 is D-Ser
  MISC_FEATURE (10)..(10): Lys10 conjugated to  gamma-Glu-gamma-Glu-C16
  MISC_FEATURE (31)..(31): Xaa31 is conjugated to  PEG2PEG2-C5N3
HXQGTFTSDKSKYLDERAAQDFVQWLLDTKK

SEQ ID NO: 97 - protein, 31 aa, Artificial Sequence; identical to SEQ ID NO: 56
  Peptide
  PEPTIDE (1)..(31): C-terminal amide
  MISC_FEATURE (2)..(2): Xaa2 is D-Ser
  MISC_FEATURE (10)..(10): Lys10 conjugated to  gamma-Glu-gamma-Glu-C16
  MISC_FEATURE (16)..(16): Xaa16 is aib
  MISC_FEATURE (24)..(24): Xaa24 is Nle(epsilon-N3)
  MISC_FEATURE (31)..(31): Xaa31 is gamma-Glu

SEQ ID NO: 98 - protein, 31 aa, Artificial Sequence
  Peptide
  PEPTIDE (1)..(31): C-terminal amide
  MISC_FEATURE (2)..(2): Xaa2 is aib
  MISC_FEATURE (10)..(10): Lys10 conjugated to  gamma-Glu-gamma-Glu-C16
  MISC_FEATURE (16)..(16): Xaa16 is aib
  MISC_FEATURE (24)..(24): Lys24 is conjugated to PEG2-C5N3
  MISC_FEATURE (31)..(31): Xaa31 is gamma-Glu
HXQGTFTSDKSKYLDXRAAQDFVKWLLDTKX

SEQ ID NO: 99 - protein, 31 aa, Artificial Sequence; identical to SEQ ID NO: 98
  Peptide
  PEPTIDE (1)..(31): C-terminal amide
  MISC_FEATURE (2)..(2): Xaa2 is aib
  MISC_FEATURE (10)..(10): Lys10 conjugated to  gamma-Glu-gamma-Glu-C16
  MISC_FEATURE (16)..(16): Xaa16 is aib
  MISC_FEATURE (24)..(24): Lys24 is conjugated to PEG2PEG2-C5N3
  MISC_FEATURE (31)..(31): Xaa31 is gamma-Glu

SEQ ID NO: 100 - protein, 29 aa, Artificial Sequence
  Peptide
  PEPTIDE (1)..(29): C-terminal amide
  MISC_FEATURE (2)..(2): Xaa2 is D-Ser
  MISC_FEATURE (10)..(10): Lys10 conjugated to  gamma-Glu-gamma-Glu-C16
  MISC_FEATURE (21)..(21): Lys21 is conjugated to  PEG2PEG2-gamma-GluC16N3
HXQGTFTSDKSKYLDERAAQKFVQWLLDT

SEQ ID NO: 101 - protein, 29 aa, Artificial Sequence
  Peptide
  PEPTIDE (1)..(29): C-terminal amide
  MISC_FEATURE (2)..(2): Xaa2 is D-Ser
  MISC_FEATURE (10)..(10): Lys10 conjugated to  gamma-Glu-gamma-Glu-C16
  MISC_FEATURE (24)..(24): Lys24 is conjugated to PEG2PEG2-gamma-glu-C16N3
HXQGTFTSDKSKYLDERAAQDFVKWLLDT

SEQ ID NO: 102 - protein, 31 aa, Artificial Sequence
  Peptide
  PEPTIDE (1)..(31): C-terminal amide
  MISC_FEATURE (2)..(2): Xaa2 is aib
  MISC_FEATURE (16)..(16): Xaa16 is aib
  MISC_FEATURE (24)..(24): Xaa24 is Nle(epsilon-N3)
HXQGTFTSDKSKYLDXRAAQDFVXWLMNTKQ

SEQ ID NO: 103 - protein, 29 aa, Artificial Sequence
  Peptide
  PEPTIDE (1)..(29): C-terminal amide
  MISC_FEATURE (2)..(2): Xaa2 is D-Ser
  MISC_FEATURE (24)..(24): Xaa24 is Nle(epsilon-N3)
HXQGTFTSDKSKYLDERAAQDFVXWLLDT

SEQ ID NO: 104 - protein, 31 aa, Artificial Sequence
  Peptide
  PEPTIDE (1)..(31): C-terminal amide
  MISC_FEATURE (2)..(2): Xaa2 is aib
  MISC_FEATURE (16)..(16): Xaa16 is aib
  MISC_FEATURE (20)..(20): Xaa20 is Nle(epsilon-N3)
HXQGTFTSDKSKYLDXRAAXDFVQWLMNTKQ

SEQ ID NO: 105 - protein, 29 aa, Artificial Sequence
  Peptide
  PEPTIDE (1)..(29): C-terminal amide
  MISC_FEATURE (2)..(2): Xaa2 is D-Ser
  MISC_FEATURE (20)..(20): Xaa20 is Nle(epsilon-N3)
HXQGTFTSDKSKYLDERAAXDFVQWLLDT

SEQ ID NO: 106 - protein, 32 aa, Artificial Sequence
  Peptide
  PEPTIDE (1)..(32): C-terminal amide
  MISC_FEATURE (2)..(2): Xaa2 is aib
  MISC_FEATURE (16)..(16): Xaa16 is aib
  MISC_FEATURE (32)..(32): Xaa32 is Nle(epsilon-N3)
HXQGTFTSDKSKYLDXRAAQDFVQWLMNTKQX

SEQ ID NO: 107 - protein, 30 aa, Artificial Sequence
  Peptide
  PEPTIDE (1)..(30): C-terminal amide
  MISC_FEATURE (2)..(2): Xaa2 is D-Ser
  MISC_FEATURE (30)..(30): Xaa30 is Nle(epsilon-N3)
HXQGTFTSDKSKYLDERAAQDFVQWLLDTX

SEQ ID NO: 108 - protein, 29 aa, Artificial Sequence
  Peptide
  PEPTIDE (1)..(29): C-terminal amide
  MISC_FEATURE (2)..(2): Xaa2 is D-Ser
  MISC_FEATURE (10)..(10): Lys10 conjugated to  gamma-Glu-gamma-Glu-C16
  MISC_FEATURE (24)..(24): Lys10 conjugated to  gamma-Glu-gamma-Glu-C16
HXQGTFTSDKSKYLDERAAQDFVXWLLDT

SEQ ID NO: 109 - protein, 29 aa, Artificial Sequence
  Peptide
  PEPTIDE (1)..(29): C-terminal amide
  MISC_FEATURE (2)..(2): Xaa2 is D-Ser
  MISC_FEATURE (10)..(10): Lys10 conjugated to  gamma-Glu-gamma-Glu-C16
  MISC_FEATURE (24)..(24): Xaa24 is Nle(epsilon-N3)
HXEGTFTSDKSKYLDERAAQDFVXWLLDT

SEQ ID NO: 110 - protein, 40 aa, Artificial Sequence
  Peptide
  PEPTIDE (1)..(40): C terminal amide
  MISC_FEATURE (40)..(40): Xaa40 is Nle(epsilonN3)
HGEGTFTSDLSKQMEEEAVRLFIEWLKNGGPSSGAPPPSX

SEQ ID NO: 111 - protein, 32 aa, Artificial Sequence
  Peptide
  MISC_FEATURE (2)..(2): Xaa2 is aib
  MISC_FEATURE (32)..(32): Xaa32 is Nle(epsilonN3)
HXEGTFTSDVSSYLEGQAAKEFIAWLVRGRGX

SEQ ID NO: 112 - protein, 32 aa, Artificial Sequence
  Peptide
  MISC_FEATURE (32)..(32): Xaa32 is Nle(epsilonN3)
HAEGTFTSDVSSYLEGQAAKEFIAWLVRGRGX

SEQ ID NO: 113 - protein, 45 aa, Artificial Sequence
  Peptide
  PEPTIDE (1)..(45): C terminal amide
  MISC_FEATURE (45)..(45): Xaa45 is Nle(epsilonN3)
HGEGTFTSKLSKQMEEEAVRLFIEWLKNGGPSSGAPPSKKKKKKX

SEQ ID NO: 114 - protein, 45 aa, Artificial Sequence
  Peptide
  PEPTIDE (1)..(45): C terminal amide
  MISC_FEATURE (45)..(45): Xaa45 is Nle(epsilonN3)
HGEGTFTSDVSSYLEEQAAKEFIAWLVKGGGGGGSGGGSGGGSAX

SEQ ID NO: 115 - protein, 30 aa, Artificial Sequence
  Peptide
  MISC_FEATURE (30)..(30): Xaa30 is Nle(epsilonN3)
HSQGTFTSDYSKYLDSRRAQDFVQWLMNTX

SEQ ID NO: 116 - protein, 43 aa, Artificial Sequence
  Peptide
  MISC_FEATURE (43)..(43): Xaa43 is Nle(epsilonN3)
YAEGTFISDYSIAMDKIHQQDFVNWLLAQKGKKNDWKHNITQX

SEQ ID NO: 117 - protein, 40 aa, Artificial Sequence
  Peptide
  PEPTIDE (1)..(40): C-terminal amide
  MISC_FEATURE (2)..(2): Xaa2 is aib
  MISC_FEATURE (20)..(20): Xaa20 is aib
  MISC_FEATURE (40)..(40): Xaa44 is Nle(epsilonN3)
YXEGTFTSDYSIYLDKQAAXEFVNWLLAGGPSSGAPPPSX

SEQ ID NO: 118 - protein, 40 aa, Artificial Sequence
  Peptide
  PEPTIDE (1)..(40): c TERMINAL AMIDE
  MISC_FEATURE (2)..(2): Xaa is aib
  MISC_FEATURE (40)..(40): Xaa40 is Nle(epsilonN3)
HXQGTFTSDKSKYLDERAAQDFVQWLLDGGPSSGAPPPSX

SEQ ID NO: 119 - protein, 38 aa, Artificial Sequence
  Peptide
  MISC_FEATURE (38)..(38): Xaa38 is Nle(epsilonN3)
HSQGTFTSDYSKYLDSRRAQDFVQWLMNTKRNKNNIAX

SEQ ID NO: 120 - protein, 37 aa, Artificial Sequence
  Peptide
  MISC_FEATURE (27)..(27): Xaa27 is Nle(epsilonN3)
HSQGTFTSDYSKYLDSRRAQDFVQWLXNTKRNKNNIA

SEQ ID NO: 121 - protein, 29 aa, Artificial Sequence
  Peptide
  PEPTIDE (1)..(29): C terminal amide
  MISC_FEATURE (2)..(2): Xaa is D-Ser
  MISC_FEATURE (10)..(10): Lys10 conjugated to gamma-Glu-gamma-Glu-C16
  MISC_FEATURE (24)..(24): Xaa24 is Nle(epsilonN3)
HXQGTFTSDKSKYLDERAAQDFVXWLLDT

SEQ ID NO: 122 - protein, 29 aa, Artificial Sequence
  Peptide
  PEPTIDE (1)..(29): C terminal amide
  MISC_FEATURE (2)..(2): Xaa is D-Ser
  MISC_FEATURE (24)..(24): Xaa24 is Nle(epsilonN3)
HXQGTFTSDKSKYLDERAAQDFVXWLLDT

SEQ ID NO: 123 - protein, 32 aa, Artificial Sequence; identical to SEQ ID NO: 106
  Peptide
  PEPTIDE (1)..(32): C terminal amide
  MISC_FEATURE (2)..(2): Xaa2 is aib
  MISC_FEATURE (10)..(10): Lys10 conjugated to gamma-Glu-gamma-Glu-C16
  MISC_FEATURE (16)..(16): Xaa16 is aib

SEQ ID NO: 124 - protein, 29 aa, Artificial Sequence
  Peptide
  PEPTIDE (1)..(29): C terminal amide
  MISC_FEATURE (2)..(2): Xaa2 is D-Ser
  MISC_FEATURE (24)..(24): Lys24 conjugated to PEG2PEG2-gamma-Glu-C16N3
HXQGTFTSDYSKYLDERAAQDFVKWLLDT

SEQ ID NO: 125 - protein, 32 aa, Artificial Sequence
  Peptide
  PEPTIDE (1)..(31): C terminal amide
  MISC_FEATURE (2)..(2): Xaa2 is aib
  MISC_FEATURE (10)..(10): Lys10 conjugated to gamma-Glu-gamma-Glu-C16
  MISC_FEATURE (16)..(16): Xaa16 is aib
  MISC_FEATURE (31)..(31): Lys31 conjugated to PEG2PEG2-C5N3
  misc_feature (32)..(32): Xaa can be any naturally occurring amino acid
HXQGTFTSDKSKYLDXRAAQDFVQWLLDTKKX

SEQ ID NO: 126 - protein, 21 aa, Homo sapiens
GIVEQCCTSICSLYQLENYCN

SEQ ID NO: 127 - protein, 30 aa, Homo sapiens
FVNQHLCGSHLVEALYLVCGERGFFYTPKT

SEQ ID NO: 128 - protein, 30 aa, Artificial Sequence
  Lispro B chain
FVNQHLCGSHLVEALYLVCGERGFFYTKPT

SEQ ID NO: 129 - protein, 30 aa, Artificial Sequence
  Aspart B chain
FVNQHLCGSHLVEALYLVCGERGFFYTDKT

SEQ ID NO: 130 - protein, 30 aa, Artificial Sequence
  Glulisine B chain
FVKQHLCGSHLVEALYLVCGERGFFYTPET

SEQ ID NO: 131 - protein, 21 aa, Artificial Sequence
  Glargine A chain
GIVEQCCTSICSLYQLENYCG

SEQ ID NO: 132 - protein, 32 aa, Artificial Sequence
  Glargine B chain
FVNQHLCGSHLVEALYLVCGERGFFYTPKTRR

SEQ ID NO: 133 - protein, 21 aa, Artificial Sequence
  Peptide
  MISC_FEATURE (8)..(8)
  MISC_FEATURE (21)..(21): Xaa is asparagine or glycine
GIVEQCCXSICSLYQLENYCX

SEQ ID NO: 134 - protein, 21 aa, Artificial Sequence
  Peptide
  MISC_FEATURE (1)..(1): Xaa is selected from the group consisting of histidine and threonine
  MISC_FEATURE (5)..(5): Xaa is selected from the group consisting of alanine, glycine and serine;
  MISC_FEATURE (6)..(6): Xaa is selected from the group consisting of histidine, aspartic acid, glutamic acid, homocysteic acid and cysteic acid
XLCGXXLVEALYLVCGERGFF

SEQ ID NO: 135 - protein, 29 aa, Artificial Sequence
  Peptide
  MISC_FEATURE (1)..(1): Xaa is selected from the group consisting of phenylalanine and desamino-phenylalanine.
  MISC_FEATURE (5)..(5): Xaa is selected from the group consisting of histidine and threonine;
  MISC_FEATURE (9)..(9): Xaa is selected from the group consisting of alanine, glycine and serine;
  MISC_FEATURE (10)..(10): Xaa is selected from the group consisting of histidine, aspartic acid, glutamic acid, homocysteic acid and cysteic acid
  misc_feature (28)..(28): Xaa can be any naturally occurring amino acid
  MISC_FEATURE (29)..(29): Xaa is threonine, alanine, or a threonine-arginine-arginine tripeptide
XVNQXLCGXXLVEALYLVCGERGFFYTXX

SEQ ID NO: 136 - protein, 22 aa, Artificial Sequence
  Peptide
  MISC_FEATURE (1)..(1): Xaa1 is glycine (G) or lysine (K)
  MISC_FEATURE (3)..(3): Xaa3 is valine (V), glycine (G), or lysine (K)
  MISC_FEATURE (5)..(5): Xaa5 is valine (V), glycine (G), or lysine (K)
  MISC_FEATURE (8)..(8): Xaa8 is threonine (T) or histidine (H)
  MISC_FEATURE (9)..(9): Xaa9 is serine (S) or lysine (K)
  MISC_FEATURE (10)..(10): Xaa10 is isoleucine (I) or lysine
  MISC_FEATURE (13)..(13): Xaa13 is leucine (L) or lysine (K)
  MISC_FEATURE (14)..(14): Xaa14 is tyrosine (Y) or lysine (K)
  MISC_FEATURE (15)..(15): Xaa15 is glutamine (Q) or lysine (K)
  MISC_FEATURE (18)..(18): Xaa18 is asparagine (N) or lysine (K)
  MISC_FEATURE (21)..(21): Xaa21 is asparagine (N) or glycine (G)
  MISC_FEATURE (22)..(22): Xaa22 is arginine (R), lysine (K) or absent
XIXEXCCXXXCSXXXLEXYCXX

SEQ ID NO: 137 - protein, 35 aa, Artificial Sequence
  Peptide
  MISC_FEATURE (1)..(1): Xaa1 is phenylalanine (F) or lysine (K)
  MISC_FEATURE (3)..(3): Xaa3 is asparagine (N) or lysine (K)
  MISC_FEATURE (4)..(4): Xaa4 is glutamine (Q) or lysine (K)
  MISC_FEATURE (16)..(16): Xaa16 is tyrosine (Y) or lysine (K)
  MISC_FEATURE (17)..(17): Xaa17 is leucine (L) or lysine (K)
  MISC_FEATURE (25)..(25): Xaa25 is phenylalanine (F) or lysine (K)
  MISC_FEATURE (28)..(28): Xaa28 is proline (P) or lysine (K)
  MISC_FEATURE (29)..(29): Xaa29 is lysine (K) or proline (P)
  MISC_FEATURE (30)..(30): Xaa30 is threonine (T) or absent
  MISC_FEATURE (31)..(31): Xaa31 is arginine (R) if Xaa30 is threonine (T), or absent
  MISC_FEATURE (32)..(32): Xaa32 is proline (P) if Xaa31 is arginine (R), or absent
  MISC_FEATURE (33)..(33): Xaa33 is arginine (R) if Xaa32 is proline (P), or absent
  MISC_FEATURE (34)..(34): Xaa34 is proline (P) if Xaa33 is arginine (R), or absent
  MISC_FEATURE (35)..(35): Xaa35 is arginine (R) if Xaa34 is proline (P), or absent
XVXXHLCGSHLVEALXXVCGERGFXYTXXXXXXXX

SEQ ID NO: 138 - protein, 29 aa, Artificial Sequence
  Peptide
  MISC_FEATURE (1)..(1): Xaa1 is phenylalanine (F) or lysine (K)
  MISC_FEATURE (3)..(3): Xaa3 is asparagine (N) or lysine (K)
  MISC_FEATURE (4)..(4): Xaa4 is glutamine (Q) or lysine (K)
  MISC_FEATURE (16)..(16): Xaa16 is tyrosine (Y) or lysine (K)
  MISC_FEATURE (17)..(17): Xaa17 is leucine (L) or lysine (K)
  MISC_FEATURE (25)..(25): Xaa25 is phenylalanine (F) or lysine (K)
  MISC_FEATURE (28)..(28): Xaa28 is proline (P) or lysine (K)
  MISC_FEATURE (29)..(29): Xaa29 is lysine (K) or proline (P)
XVXXHLCGSHLVEALXXVCGERGFXYTXX

SEQ ID NO: 139 - protein, 35 aa, Artificial Sequence
  Peptide
  MISC_FEATURE (1)..(1): Xaa1 is phenylalanine (F) or lysine (K)
  MISC_FEATURE (3)..(3): Xaa3 is asparagine (N) or lysine (K)
  MISC_FEATURE (4)..(4): Xaa4 is glutamine (Q) or lysine (K)
  MISC_FEATURE (16)..(16): Xaa16 is tyrosine (Y) or lysine (K)
  MISC_FEATURE (17)..(17): Xaa17 is leucine (L) or lysine (K)
  MISC_FEATURE (25)..(25): Xaa25 is phenylalanine (F) or lysine (K)
  MISC_FEATURE (28)..(28): Xaa28 is proline (P) or lysine (K)
  MISC_FEATURE (29)..(29): Xaa29 is lysine (K) or proline (P)
XVXXHLCGSHLVEALXXVCGERGFXYTXXTRPRPR

SEQ ID NO: 140 - protein, 33 aa, Artificial Sequence
  Peptide
  MISC_FEATURE (1)..(1): Xaa1 is phenylalanine (F) or lysine (K)
  MISC_FEATURE (3)..(3): Xaa3 is asparagine (N) or lysine (K)
  MISC_FEATURE (4)..(4): Xaa4 is glutamine (Q) or lysine (K)
  MISC_FEATURE (16)..(16): Xaa16 is tyrosine (Y) or lysine (K)
  MISC_FEATURE (17)..(17): Xaa17 is leucine (L) or lysine (K)
  MISC_FEATURE (25)..(25): Xaa25 is phenylalanine (F) or lysine (K)
  MISC_FEATURE (28)..(28): Xaa28 is proline (P) or lysine (K)
  MISC_FEATURE (29)..(29): Xaa29 is lysine (K) or proline (P)
XVXXHLCGSHLVEALXXVCGERGFXYTXXTRPR

SEQ ID NO: 141 - protein, 29 aa, Artificial Sequence
  Petide
  PEPTIDE (1)..(29): C terminal amide
  MISC_FEATURE (2)..(2): Xaa2 is D-Ser
  MISC_FEATURE (10)..(10): Lys10 conjugated to gamma-Glu-gamma-Glu-C16
HXQGTFTSDKSKYLDERAAQDFVQWLLDT